European Patent Application EP 4 477 754 A2, published December 18, 2024. Title: TaRGET SYSTEM FOR HOMOLOGY-DIRECTED REPAIR AND GENE EDITING METHOD USING THE SAME. Applicant: 주식회사 진코어. The sequence listing filed with the application follows.

SEQUENCE LISTING (302 sequences)

SEQ ID NO: 1 - protein, 557 aa, unidentified
  source 1..557: note = TnpB
MGEKSSRRRRNGKSGAWTAAITSCVGGKMAKNTITKTLKLRIVRPYNSAEVEKIVADEKNNREKIALEKNKDKVKEACSKHLKVAAYCTTQVERNACLFCKARKLDDKFYQKLRGQFPDAVFWQEISEIFRQLQKQAAEIYNQSLIELYYEIFIKGKGIANASSVEHYLSDVCYTRAAELFKNAAIASGLRSKIKSNFRLKELKNMKSGLPTTKSDNFPIPLVKQKGGQYTGFEISNHNSDFIIKIPFGRWQVKKEIDKYRPWEKFDFEQVQKSPKPISLLLSTQRRKRNKGWSKDEGTEAEIKKVMNGDYQTSYIEVKRGSKIGEKSAWMLNLSIDVPKIDKGVDPSIIGGIDVGVKSPLVCAINNAFSRYSISDNDLFHFNKKMFARRRILLKKNRHKRAGHGAKNKLKPITILTEKSERFRKKLIERWACEIADFFIKNKVGTVQMENLESMKRKEDSYFNIRLRGFWPYAEMQNKIEFKLKQYGIEIRKVAPNNTSKTCSKCGHLNNYFNFEYRKKNKFPHFKCEKCNFKENADYNAALNISNPKLKSTKEEP

SEQ ID NO: 2 - protein, 555 aa, synthetic construct
  source 1..555: note = TnpB-v1
MEKRINKIRKKLSADNATKPVSRSGPMAKNTITKTLKLRIVRPYNSAEVEKIVADEKNNREKIALEKNKDKVKEACSKHLKVAAYCTTQVERNACLFCKARKLDDKFYQKLRGQFPDAVFWQEISEIFRQLQKQAAEIYNQSLIELYYEIFIKGKGIANASSVEHYLSDVCYTRAAELFKNAAIASGLRSKIKSNFRLKELKNMKSGLPTTKSDNFPIPLVKQKGGQYTGFEISNHNSDFIIKIPFGRWQVKKEIDKYRPWEKFDFEQVQKSPKPISLLLSTQRRKRNKGWSKDEGTEAEIKKVMNGDYQTSYIEVKRGSKIGEKSAWMLNLSIDVPKIDKGVDPSIIGGIDVGVKSPLVCAINNAFSRYSISDNDLFHFNKKMFARRRILLKKNRHKRAGHGAKNKLKPITILTEKSERFRKKLIERWACEIADFFIKNKVGTVQMENLESMKRKEDSYFNIRLRGFWPYAEMQNKIEFKLKQYGIEIRKVAPNNTSKTCSKCGHLNNYFNFEYRKKNKFPHFKCEKCNFKENADYNAALNISNPKLKSTKEEP

SEQ ID NO: 3 - protein, 557 aa, synthetic construct
  source 1..557: note = TnpB-v2
MAGGPGAGSAAPVSSTSSLPLAALNMRVMAKNTITKTLKLRIVRPYNSAEVEKIVADEKNNREKIALEKNKDKVKEACSKHLKVAAYCTTQVERNACLFCKARKLDDKFYQKLRGQFPDAVFWQEISEIFRQLQKQAAEIYNQSLIELYYEIFIKGKGIANASSVEHYLSDVCYTRAAELFKNAAIASGLRSKIKSNFRLKELKNMKSGLPTTKSDNFPIPLVKQKGGQYTGFEISNHNSDFIIKIPFGRWQVKKEIDKYRPWEKFDFEQVQKSPKPISLLLSTQRRKRNKGWSKDEGTEAEIKKVMNGDYQTSYIEVKRGSKIGEKSAWMLNLSIDVPKIDKGVDPSIIGGIDVGVKSPLVCAINNAFSRYSISDNDLFHFNKKMFARRRILLKKNRHKRAGHGAKNKLKPITILTEKSERFRKKLIERWACEIADFFIKNKVGTVQMENLESMKRKEDSYFNIRLRGFWPYAEMQNKIEFKLKQYGIEIRKVAPNNTSKTCSKCGHLNNYFNFEYRKKNKFPHFKCEKCNFKENADYNAALNISNPKLKSTKEEP

SEQ ID NO: 4 - protein, 555 aa, synthetic construct
  source 1..555: note = TnpB-v3
MAGGPGAGSAAPVSSTSSLPLAALNMMAKNTITKTLKLRIVRPYNSAEVEKIVADEKNNREKIALEKNKDKVKEACSKHLKVAAYCTTQVERNACLFCKARKLDDKFYQKLRGQFPDAVFWQEISEIFRQLQKQAAEIYNQSLIELYYEIFIKGKGIANASSVEHYLSDVCYTRAAELFKNAAIASGLRSKIKSNFRLKELKNMKSGLPTTKSDNFPIPLVKQKGGQYTGFEISNHNSDFIIKIPFGRWQVKKEIDKYRPWEKFDFEQVQKSPKPISLLLSTQRRKRNKGWSKDEGTEAEIKKVMNGDYQTSYIEVKRGSKIGEKSAWMLNLSIDVPKIDKGVDPSIIGGIDVGVKSPLVCAINNAFSRYSISDNDLFHFNKKMFARRRILLKKNRHKRAGHGAKNKLKPITILTEKSERFRKKLIERWACEIADFFIKNKVGTVQMENLESMKRKEDSYFNIRLRGFWPYAEMQNKIEFKLKQYGIEIRKVAPNNTSKTCSKCGHLNNYFNFEYRKKNKFPHFKCEKCNFKENADYNAALNISNPKLKSTKEEP

SEQ ID NO: 5 - protein, 529 aa, synthetic construct
  source 1..529: note = Wild-type Cas12f1
MAKNTITKTLKLRIVRPYNSAEVEKIVADEKNNREKIALEKNKDKVKEACSKHLKVAAYCTTQVERNACLFCKARKLDDKFYQKLRGQFPDAVFWQEISEIFRQLQKQAAEIYNQSLIELYYEIFIKGKGIANASSVEHYLSDVCYTRAAELFKNAAIASGLRSKIKSNFRLKELKNMKSGLPTTKSDNFPIPLVKQKGGQYTGFEISNHNSDFIIKIPFGRWQVKKEIDKYRPWEKFDFEQVQKSPKPISLLLSTQRRKRNKGWSKDEGTEAEIKKVMNGDYQTSYIEVKRGSKIGEKSAWMLNLSIDVPKIDKGVDPSIIGGIDVGVKSPLVCAINNAFSRYSISDNDLFHFNKKMFARRRILLKKNRHKRAGHGAKNKLKPITILTEKSERFRKKLIERWACEIADFFIKNKVGTVQMENLESMKRKEDSYFNIRLRGFWPYAEMQNKIEFKLKQYGIEIRKVAPNNTSKTCSKCGHLNNYFNFEYRKKNKFPHFKCEKCNFKENADYNAALNISNPKLKSTKEEP

SEQ ID NO: 6 - DNA, 1671 bp, synthetic construct
  source 1..1671: mol_type = other DNA; note = Human codon-optimized TnpB
atgggggagaaaagttcccgccgccgacggaatggaaaaagcggtgcgtggactgctgctataacaagctgtgttgggggtaagatggccaagaacacaattacaaagacactgaagctgaggatcgtgagaccatacaacagcgctgaggtcgagaagattgtggctgatgaaaagaacaacagggaaaagatcgccctcgagaagaacaaggataaggtgaaggaggcctgctctaagcacctgaaagtggccgcctactgcaccacacaggtggagaggaacgcctgtctgttttgtaaagctcggaagctggatgataagttttaccagaagctgcggggccagttccccgatgccgtcttttggcaggagattagcgagatcttcagacagctgcagaagcaggccgccgagatctacaaccagagcctgatcgagctctactacgagatcttcatcaagggcaagggcattgccaacgcctcctccgtggagcactacctgagcgacgtgtgctacacaagagccgccgagctctttaagaacgccgctatcgcttccgggctgaggagcaagattaagagtaacttccggctcaaggagctgaagaacatgaagagcggcctgcccactacaaagagcgacaacttcccaattccactggtgaagcagaaggggggccagtacacagggttcgagatttccaaccacaacagcgactttattattaagatcccctttggcaggtggcaggtcaagaaggagattgacaagtacaggccctgggagaagtttgatttcgagcaggtgcagaagagccccaagcctatttccctgctgctgtccacacagcggcggaagaggaacaaggggtggtctaaggatgaggggaccgaggccgagattaagaaagtgatgaacggcgactaccagacaagctacatcgaggtcaagcggggcagtaagattggcgagaagagcgcctggatgctgaacctgagcattgacgtgccaaagattgataagggcgtggatcccagcatcatcggagggatcgatgtgggggtcaagagccccctcgtgtgcgccatcaacaacgccttcagcaggtacagcatctccgataacgacctgttccactttaacaagaagatgttcgcccggcggaggattttgctcaagaagaaccggcacaagcgggccggacacggggccaagaacaagctcaagcccatcactatcctgaccgagaagagcgagaggttcaggaagaagctcatcgagagatgggcctgcgagatcgccgatttctttattaagaacaaggtcggaacagtgcagatggagaacctcgagagcatgaagaggaaggaggattcctacttcaacattcggctgagggggttctggccctacgctgagatgcagaacaagattgagtttaagctgaagcagtacgggattgagatccggaaggtggcccccaacaacaccagcaagacctgcagcaagtgcgggcacctcaacaactacttcaacttcgagtaccggaagaagaacaagttcccacacttcaagtgcgagaagtgcaactttaaggagaacgccgattacaacgccgccctgaacatcagcaaccctaagctgaagagcactaaggaggagccc

SEQ ID NO: 7 - DNA, 1666 bp, synthetic construct
  source 1..1666: mol_type = other DNA; note = Human codon-optimized TnpB-V1
atggaaaagagaatcaacaagatcaggaagaagctgagcgccgacaacgccaccaagcctgtgtctaggagtggcccccatggccaagaacacaattacaaagacactgaagctgaggatcgtgagaccatacaacagcgctgaggtcgagaagattgtggctgatgaaaagaacaacagggaaaagatcgccctcgagaagaacaaggataaggtgaaggaggcctgctctaagcacctgaaagtggccgcctactgcaccacacaggtggagaggaacgcctgtctgttttgtaaagctcggaagctggatgataagttttaccagaagctgcggggccagttccccgatgccgtcttttggcaggagattagcgagatcttcagacagctgcagaagcaggccgccgagatctacaaccagagcctgatcgagctctactacgagatcttcatcaagggcaagggcattgccaacgcctcctccgtggagcactacctgagcgacgtgtgctacacaagagccgccgagctctttaagaacgccgctatcgcttccgggctgaggagcaagattaagagtaacttccggctcaaggagctgaagaacatgaagagcggcctgcccactacaaagagcgacaacttcccaattccactggtgaagcagaaggggggccagtacacagggttcgagatttccaaccacaacagcgactttattattaagatcccctttggcaggtggcaggtcaagaaggagattgacaagtacaggccctgggagaagtttgatttcgagcaggtgcagaagagccccaagcctatttccctgctgctgtccacacagcggcggaagaggaacaaggggtggtctaaggatgaggggaccgaggccgagattaagaaagtgatgaacggcgactaccagacaagctacatcgaggtcaagcggggcagtaagattggcgagaagagcgcctggatgctgaacctgagcattgacgtgccaaagattgataagggcgtggatcccagcatcatcggagggatcgatgtgggggtcaagagccccctcgtgtgcgccatcaacaacgccttcagcaggtacagcatctccgataacgacctgttccactttaacaagaagatgttcgcccggcggaggattttgctcaagaagaaccggcacaagcgggccggacacggggccaagaacaagctcaagcccatcactatcctgaccgagaagagcgagaggttcaggaagaagctcatcgagagatgggcctgcgagatcgccgatttctttattaagaacaaggtcggaacagtgcagatggagaacctcgagagcatgaagaggaaggaggattcctacttcaacattcggctgagggggttctggccctacgctgagatgcagaacaagattgagtttaagctgaagcagtacgggattgagatccggaaggtggcccccaacaacaccagcaagacctgcagcaagtgcgggcacctcaacaactacttcaacttcgagtaccggaagaagaacaagttcccacacttcaagtgcgagaagtgcaactttaaggagaacgccgattacaacgccgccctgaacatcagcaaccctaagctgaagagcactaaggaggagccc

SEQ ID NO: 8 - DNA, 1671 bp, synthetic construct
  source 1..1671: mol_type = other DNA; note = Human codon-optimized TnpB-V2
atggctggcggaccaggcgcaggtagtgctgcgccagtttcttcaacttcctccctgcccctggctgcgcttaacatgcgcgtgatggccaagaacacaattacaaagacactgaagctgaggatcgtgagaccatacaacagcgctgaggtcgagaagattgtggctgatgaaaagaacaacagggaaaagatcgccctcgagaagaacaaggataaggtgaaggaggcctgctctaagcacctgaaagtggccgcctactgcaccacacaggtggagaggaacgcctgtctgttttgtaaagctcggaagctggatgataagttttaccagaagctgcggggccagttccccgatgccgtcttttggcaggagattagcgagatcttcagacagctgcagaagcaggccgccgagatctacaaccagagcctgatcgagctctactacgagatcttcatcaagggcaagggcattgccaacgcctcctccgtggagcactacctgagcgacgtgtgctacacaagagccgccgagctctttaagaacgccgctatcgcttccgggctgaggagcaagattaagagtaacttccggctcaaggagctgaagaacatgaagagcggcctgcccactacaaagagcgacaacttcccaattccactggtgaagcagaaggggggccagtacacagggttcgagatttccaaccacaacagcgactttattattaagatcccctttggcaggtggcaggtcaagaaggagattgacaagtacaggccctgggagaagtttgatttcgagcaggtgcagaagagccccaagcctatttccctgctgctgtccacacagcggcggaagaggaacaaggggtggtctaaggatgaggggaccgaggccgagattaagaaagtgatgaacggcgactaccagacaagctacatcgaggtcaagcggggcagtaagattggcgagaagagcgcctggatgctgaacctgagcattgacgtgccaaagattgataagggcgtggatcccagcatcatcggagggatcgatgtgggggtcaagagccccctcgtgtgcgccatcaacaacgccttcagcaggtacagcatctccgataacgacctgttccactttaacaagaagatgttcgcccggcggaggattttgctcaagaagaaccggcacaagcgggccggacacggggccaagaacaagctcaagcccatcactatcctgaccgagaagagcgagaggttcaggaagaagctcatcgagagatgggcctgcgagatcgccgatttctttattaagaacaaggtcggaacagtgcagatggagaacctcgagagcatgaagaggaaggaggattcctacttcaacattcggctgagggggttctggccctacgctgagatgcagaacaagattgagtttaagctgaagcagtacgggattgagatccggaaggtggcccccaacaacaccagcaagacctgcagcaagtgcgggcacctcaacaactacttcaacttcgagtaccggaagaagaacaagttcccacacttcaagtgcgagaagtgcaactttaaggagaacgccgattacaacgccgccctgaacatcagcaaccctaagctgaagagcactaaggaggagccc

SEQ ID NO: 9 - DNA, 1665 bp, synthetic construct
  source 1..1665: mol_type = other DNA; note = Human codon-optimized TnpB-V3
atggctggcggaccaggcgcaggtagtgctgcgccagtttcttcaacttcctccctgcccctggctgcgcttaacatgatggccaagaacacaattacaaagacactgaagctgaggatcgtgagaccatacaacagcgctgaggtcgagaagattgtggctgatgaaaagaacaacagggaaaagatcgccctcgagaagaacaaggataaggtgaaggaggcctgctctaagcacctgaaagtggccgcctactgcaccacacaggtggagaggaacgcctgtctgttttgtaaagctcggaagctggatgataagttttaccagaagctgcggggccagttccccgatgccgtcttttggcaggagattagcgagatcttcagacagctgcagaagcaggccgccgagatctacaaccagagcctgatcgagctctactacgagatcttcatcaagggcaagggcattgccaacgcctcctccgtggagcactacctgagcgacgtgtgctacacaagagccgccgagctctttaagaacgccgctatcgcttccgggctgaggagcaagattaagagtaacttccggctcaaggagctgaagaacatgaagagcggcctgcccactacaaagagcgacaacttcccaattccactggtgaagcagaaggggggccagtacacagggttcgagatttccaaccacaacagcgactttattattaagatcccctttggcaggtggcaggtcaagaaggagattgacaagtacaggccctgggagaagtttgatttcgagcaggtgcagaagagccccaagcctatttccctgctgctgtccacacagcggcggaagaggaacaaggggtggtctaaggatgaggggaccgaggccgagattaagaaagtgatgaacggcgactaccagacaagctacatcgaggtcaagcggggcagtaagattggcgagaagagcgcctggatgctgaacctgagcattgacgtgccaaagattgataagggcgtggatcccagcatcatcggagggatcgatgtgggggtcaagagccccctcgtgtgcgccatcaacaacgccttcagcaggtacagcatctccgataacgacctgttccactttaacaagaagatgttcgcccggcggaggattttgctcaagaagaaccggcacaagcgggccggacacggggccaagaacaagctcaagcccatcactatcctgaccgagaagagcgagaggttcaggaagaagctcatcgagagatgggcctgcgagatcgccgatttctttattaagaacaaggtcggaacagtgcagatggagaacctcgagagcatgaagaggaaggaggattcctacttcaacattcggctgagggggttctggccctacgctgagatgcagaacaagattgagtttaagctgaagcagtacgggattgagatccggaaggtggcccccaacaacaccagcaagacctgcagcaagtgcgggcacctcaacaactacttcaacttcgagtaccggaagaagaacaagttcccacacttcaagtgcgagaagtgcaactttaaggagaacgccgattacaacgccgccctgaacatcagcaaccctaagctgaagagcactaaggaggagccc

SEQ ID NO: 10 - DNA, 1587 bp, synthetic construct
  source 1..1587: mol_type = other DNA; note = Human codon-optimized Cas12f1
atggccaagaacacaattacaaagacactgaagctgaggatcgtgagaccatacaacagcgctgaggtcgagaagattgtggctgatgaaaagaacaacagggaaaagatcgccctcgagaagaacaaggataaggtgaaggaggcctgctctaagcacctgaaagtggccgcctactgcaccacacaggtggagaggaacgcctgtctgttttgtaaagctcggaagctggatgataagttttaccagaagctgcggggccagttccccgatgccgtcttttggcaggagattagcgagatcttcagacagctgcagaagcaggccgccgagatctacaaccagagcctgatcgagctctactacgagatcttcatcaagggcaagggcattgccaacgcctcctccgtggagcactacctgagcgacgtgtgctacacaagagccgccgagctctttaagaacgccgctatcgcttccgggctgaggagcaagattaagagtaacttccggctcaaggagctgaagaacatgaagagcggcctgcccactacaaagagcgacaacttcccaattccactggtgaagcagaaggggggccagtacacagggttcgagatttccaaccacaacagcgactttattattaagatcccctttggcaggtggcaggtcaagaaggagattgacaagtacaggccctgggagaagtttgatttcgagcaggtgcagaagagccccaagcctatttccctgctgctgtccacacagcggcggaagaggaacaaggggtggtctaaggatgaggggaccgaggccgagattaagaaagtgatgaacggcgactaccagacaagctacatcgaggtcaagcggggcagtaagattggcgagaagagcgcctggatgctgaacctgagcattgacgtgccaaagattgataagggcgtggatcccagcatcatcggagggatcgatgtgggggtcaagagccccctcgtgtgcgccatcaacaacgccttcagcaggtacagcatctccgataacgacctgttccactttaacaagaagatgttcgcccggcggaggattttgctcaagaagaaccggcacaagcgggccggacacggggccaagaacaagctcaagcccatcactatcctgaccgagaagagcgagaggttcaggaagaagctcatcgagagatgggcctgcgagatcgccgatttctttattaagaacaaggtcggaacagtgcagatggagaacctcgagagcatgaagaggaaggaggattcctacttcaacattcggctgagggggttctggccctacgctgagatgcagaacaagattgagtttaagctgaagcagtacgggattgagatccggaaggtggcccccaacaacaccagcaagacctgcagcaagtgcgggcacctcaacaactacttcaacttcgagtaccggaagaagaacaagttcccacacttcaagtgcgagaagtgcaactttaaggagaacgccgattacaacgccgccctgaacatcagcaaccctaagctgaagagcactaaggaggagccc

SEQ ID NO: 11 - RNA, 161 nt, synthetic construct
  source 1..161: mol_type = other RNA; note = Wild-type tracrRNA for TnpB gRNA
cttcactgataaagtggagaaccgcttcaccaaaagctgtcccttaggggattagaacttgagtgaaggtgggctgcttgcatcagcctaatgtcgagaagtgctttcttcggaaagtaaccctcgaaacaaattcatttttcctctccaattctgcacaa

SEQ ID NO: 12 - RNA, 37 nt, synthetic construct
  source 1..37: mol_type = other RNA; note = Wild-type crRNA for TnpB gRNA
gttgcagaacccgaatagacgaatgaaggaatgcaac

SEQ ID NO: 13 - RNA, 222 nt, synthetic construct
  source 1..222: mol_type = other RNA; note = Canonical sgRNA forTnpB
  misc_feature 203..222: note = n is a, c, g or u
cttcactgataaagtggagaaccgcttcaccaaaagctgtcccttaggggattagaacttgagtgaaggtgggctgcttgcatcagcctaatgtcgagaagtgctttcttcggaaagtaaccctcgaaacaaattcatttttcctctccaattctgcacaagaaagttgcagaacccgaatagacgaatgaaggaatgcaacnnnnnnnnnnnnnnnnnnnn

SEQ ID NO: 14 - RNA, 20 nt, synthetic construct
  source 1..20: mol_type = other RNA; note = Xa of Formula (I)
cttcactgataaagtggaga

SEQ ID NO: 15 - RNA, 19 nt, synthetic construct
  source 1..19: mol_type = other RNA; note = Xa of Formula (I)
ttcactgataaagtggaga

SEQ ID NO: 16 - RNA, 18 nt, synthetic construct
  source 1..18: mol_type = other RNA; note = Xa of Formula (I)
tcactgataaagtggaga

SEQ ID NO: 17 - RNA, 17 nt, synthetic construct
  source 1..17: mol_type = other RNA; note = Xa of Formula (I)
cactgataaagtggaga

SEQ ID NO: 18 - RNA, 16 nt, synthetic construct
  source 1..16: mol_type = other RNA; note = Xa of Formula (I)
actgataaagtggaga

SEQ ID NO: 19 - RNA, 15 nt, synthetic construct
  source 1..15: mol_type = other RNA; note = Xa of Formula (I)
ctgataaagtggaga

SEQ ID NO: 20 - RNA, 14 nt, synthetic construct
  source 1..14: mol_type = other RNA; note = Xa of Formula (I)
tgataaagtggaga

SEQ ID NO: 21 - RNA, 13 nt, synthetic construct
  source 1..13: mol_type = other RNA; note = Xa of Formula (I)
gataaagtggaga

SEQ ID NO: 22 - RNA, 12 nt, synthetic construct
  source 1..12: mol_type = other RNA; note = Xa of Formula (I)
ataaagtggaga

SEQ ID NO: 23 - RNA, 11 nt, synthetic construct
  source 1..11: mol_type = other RNA; note = Xa of Formula (I)
taaagtggaga

SEQ ID NO: 24 - RNA, 10 nt, synthetic construct
  source 1..10: mol_type = other RNA; note = Xa of Formula (I)
aaagtggaga

SEQ ID NO: 25 - RNA, 13 nt, synthetic construct
  source 1..13: mol_type = other RNA; note = Xb1 of Formula (I)
caaaagctgtccc

SEQ ID NO: 26 - RNA, 12 nt, synthetic construct
  source 1..12: mol_type = other RNA; note = Xb1 of Formula (I)
caaaagctgtcc

SEQ ID NO: 27 - RNA, 11 nt, synthetic construct
  source 1..11: mol_type = other RNA; note = Xb1 of Formula (I)
caaaagctgtc

SEQ ID NO: 28 - RNA, 10 nt, synthetic construct
  source 1..10: mol_type = other RNA; note = Xb1 of Formula (I)
caaaagctgt

SEQ ID NO: 29 - RNA, 14 nt, synthetic construct
  source 1..14: mol_type = other RNA; note = Xb2 of Formula (I)
gggattagaacttg

SEQ ID NO: 30 - RNA, 13 nt, synthetic construct
  source 1..13: mol_type = other RNA; note = Xb2 of Formula (I)
ggattagaacttg

SEQ ID NO: 31 - RNA, 12 nt, synthetic construct
  source 1..12: mol_type = other RNA; note = Xb2 of Formula (I)
gattagaacttg

SEQ ID NO: 32 - RNA, 11 nt, synthetic construct
  source 1..11: mol_type = other RNA; note = Xb2 of Formula (I)
attagaacttg

SEQ ID NO: 33 - RNA, 10 nt, synthetic construct
  source 1..10: mol_type = other RNA; note = Xb2 of Formula (I)
ttagaacttg

SEQ ID NO: 34 - RNA, 31 nt, synthetic construct
  source 1..31: mol_type = other RNA; note = Xb1-UUAG-Xb2 of Formula (I)
caaaagctgtcccttaggggattagaacttg

SEQ ID NO: 35 - RNA, 25 nt, synthetic construct
  source 1..25: mol_type = other RNA; note = Xb1-UUAG-Xb2 of Formula (I)
caaaagctgtttagattagaacttg

SEQ ID NO: 36 - RNA, 20 nt, synthetic construct
  source 1..20: mol_type = other RNA; note = Xb1-UUAG-Xb2 of Formula (I)
caaaagctttagagaacttg

SEQ ID NO: 37 - RNA, 18 nt, synthetic construct
  source 1..18: mol_type = other RNA; note = Xb1-UUAG-Xb2 of Formula (I)
caaaagcttaggaacttg

SEQ ID NO: 38 - RNA, 10 nt, synthetic construct
  source 1..10: mol_type = other RNA; note = Xb1-UUAG-Xb2 of Formula (I)
caattagttg

SEQ ID NO: 39 - RNA, 28 nt, synthetic construct
  source 1..28: mol_type = other RNA; note = Xc1 of Formula (I)
ttcatttttcctctccaattctgcacaa

SEQ ID NO: 40 - RNA, 27 nt, synthetic construct
  source 1..27: mol_type = other RNA; note = Xc1 of Formula (I)
ttcatttttcctctccaattctgcaca

SEQ ID NO: 41 - RNA, 26 nt, synthetic construct
  source 1..26: mol_type = other RNA; note = Xc1 of Formula (I)
ttcatttttcctctccaattctgcac

SEQ ID NO: 42 - RNA, 25 nt, synthetic construct
  source 1..25: mol_type = other RNA; note = Xc1 of Formula (I)
ttcatttttcctctccaattctgca

SEQ ID NO: 43 - RNA, 24 nt, synthetic construct
  source 1..24: mol_type = other RNA; note = Xc1 of Formula (I)
ttcatttttcctctccaattctgc

SEQ ID NO: 44 - RNA, 23 nt, synthetic construct
  source 1..23: mol_type = other RNA; note = Xc1 of Formula (I)
ttcatttttcctctccaattctg

SEQ ID NO: 45 - RNA, 22 nt, synthetic construct
  source 1..22: mol_type = other RNA; note = Xc1 of Formula (I)
ttcatttttcctctccaattct

SEQ ID NO: 46 - RNA, 21 nt, synthetic construct
  source 1..21: mol_type = other RNA; note = Xc1 of Formula (I)
ttcatttttcctctccaattc

SEQ ID NO: 47 - RNA, 20 nt, synthetic construct
  source 1..20: mol_type = other RNA; note = Xc1 of Formula (I)
ttcatttttcctctccaatt

SEQ ID NO: 48 - RNA, 19 nt, synthetic construct
  source 1..19: mol_type = other RNA; note = Xc1 of Formula (I)
ttcatttttcctctccaat

SEQ ID NO: 49 - RNA, 18 nt, synthetic construct
  source 1..18: mol_type = other RNA; note = Xc1 of Formula (I)
ttcatttttcctctccaa

SEQ ID NO: 50 - RNA, 17 nt, synthetic construct
  source 1..17: mol_type = other RNA; note = Xc1 of Formula (I)
ttcatttttcctctcca

SEQ ID NO: 51 - RNA, 16 nt, synthetic construct
  source 1..16: mol_type = other RNA; note = Xc1 of Formula (I)
ttcatttttcctctcc

SEQ ID NO: 52 - RNA, 15 nt, synthetic construct
  source 1..15: mol_type = other RNA; note = Xc1 of Formula (I)
ttcatttttcctctc

SEQ ID NO: 53 - RNA, 14 nt, synthetic construct
  source 1..14: mol_type = other RNA; note = Xc1 of Formula (I)
ttcatttttcctct

SEQ ID NO: 54 - RNA, 13 nt, synthetic construct
  source 1..13: mol_type = other RNA; note = Xc1 of Formula (I)
ttcatttttcctc

SEQ ID NO: 55 - RNA, 12 nt, synthetic construct
  source 1..12: mol_type = other RNA; note = Xc1 of Formula (I)
ttcatttttcct

SEQ ID NO: 56 - RNA, 11 nt, synthetic construct
  source 1..11: mol_type = other RNA; note = Xc1 of Formula (I)
ttcatttttcc

SEQ ID NO: 57 - RNA, 10 nt, synthetic construct
  source 1..10: mol_type = other RNA; note = Xc1 of Formula (I)
ttcatttttc

SEQ ID NO: 58 - RNA, 27 nt, synthetic construct
  source 1..27: mol_type = other RNA; note = Xc2 of Formula (I)
gttgcagaacccgaatagacgaatgaa

SEQ ID NO: 59 - RNA, 26 nt, synthetic construct
  source 1..26: mol_type = other RNA; note = Xc2 of Formula (I)
ttgcagaacccgaatagacgaatgaa

SEQ ID NO: 60 - RNA, 25 nt, synthetic construct
  source 1..25: mol_type = other RNA; note = Xc2 of Formula (I)
tgcagaacccgaatagacgaatgaa

SEQ ID NO: 61 - RNA, 24 nt, synthetic construct
  source 1..24: mol_type = other RNA; note = Xc2 of Formula (I)
gcagaacccgaatagacgaatgaa

SEQ ID NO: 62 - RNA, 23 nt, synthetic construct
  source 1..23: mol_type = other RNA; note = Xc2 of Formula (I)
cagaacccgaatagacgaatgaa

SEQ ID NO: 63 - RNA, 22 nt, synthetic construct
  source 1..22: mol_type = other RNA; note = Xc2 of Formula (I)
agaacccgaatagacgaatgaa

SEQ ID NO: 64 - RNA, 21 nt, synthetic construct
  source 1..21: mol_type = other RNA; note = Xc2 of Formula (I)
gaacccgaatagacgaatgaa

SEQ ID NO: 65 - RNA, 20 nt, synthetic construct
  source 1..20: mol_type = other RNA; note = Xc2 of Formula (I)
aacccgaatagacgaatgaa

SEQ ID NO: 66 - RNA, 19 nt, synthetic construct
  source 1..19: mol_type = other RNA; note = Xc2 of Formula (I)
acccgaatagacgaatgaa

SEQ ID NO: 67 - RNA, 18 nt, synthetic construct
  source 1..18: mol_type = other RNA; note = Xc2 of Formula (I)
cccgaatagacgaatgaa

SEQ ID NO: 68 - RNA, 17 nt, synthetic construct
  source 1..17: mol_type = other RNA; note = Xc2 of Formula (I)
ccgaatagacgaatgaa

SEQ ID NO: 69 - RNA, 16 nt, synthetic construct
  source 1..16: mol_type = other RNA; note = Xc2 of Formula (I)
cgaatagacgaatgaa

SEQ ID NO: 70 - RNA, 15 nt, synthetic construct
  source 1..15: mol_type = other RNA; note = Xc2 of Formula (I)
gaatagacgaatgaa

SEQ ID NO: 71 - RNA, 14 nt, synthetic construct
  source 1..14: mol_type = other RNA; note = Xc2 of Formula (I)
aatagacgaatgaa

SEQ ID NO: 72 - RNA, 13 nt, synthetic construct
  source 1..13: mol_type = other RNA; note = Xc2 of Formula (I)
atagacgaatgaa

SEQ ID NO: 73 - RNA, 12 nt, synthetic construct
  source 1..12: mol_type = other RNA; note = Xc2 of Formula (I)
tagacgaatgaa

SEQ ID NO: 74 - RNA, 11 nt, synthetic construct
  source 1..11: mol_type = other RNA; note = Xc2 of Formula (I)
agacgaatgaa

SEQ ID NO: 75 - RNA, 10 nt, synthetic construct
  source 1..10: mol_type = other RNA; note = Xc2 of Formula (I)
gacgaatgaa

SEQ ID NO: 76 - RNA, 10 nt, synthetic construct
  source 1..10: mol_type = other RNA; note = Linker (Lk)
ttcgaaagaa

SEQ ID NO: 77 - RNA, 12 nt, synthetic construct
  source 1..12: mol_type = other RNA; note = Linker (Lk)
ttcagaaatgaa

SEQ ID NO: 78 - RNA, 14 nt, synthetic construct
  source 1..14: mol_type = other RNA; note = Linker (Lk)
ttcatgaaaatgaa

SEQ ID NO: 79 - RNA, 16 nt, synthetic construct
  source 1..16: mol_type = other RNA; note = Linker (Lk)
ttcattgaaaaatgaa

SEQ ID NO: 80 - RNA, 59 nt, synthetic construct
  source 1..59: mol_type = other RNA; note = Xc1-Lk-Xc2 of Formula (I)
ttcagtgctcctctccaattctgcacaagaaagttgcagaacccgaatagagcaatgaa

SEQ ID NO: 81 - RNA, 46 nt, synthetic construct
  source 1..46: mol_type = other RNA; note = Xc1-Lk-Xc2 of Formula (I)
ttcagtgctcctctccaattcgaaagaacccgaatagagcaatgaa

SEQ ID NO: 82 - RNA, 34 nt, synthetic construct
  source 1..34: mol_type = other RNA; note = Xc1-Lk-Xc2 of Formula (I)
ttcagtgctcctctcgaaagaatagagcaatgaa

SEQ ID NO: 83 - RNA, 22 nt, synthetic construct
  source 1..22: mol_type = other RNA; note = Xc1-Lk-Xc2 of Formula (I)
ttcagtgctgaaaagcaatgaa

SEQ ID NO: 84 - RNA, 18 nt, synthetic construct
  source 1..18: mol_type = other RNA; note = Xc1-Lk-Xc2 of Formula (I)
ttcatttgaaagaatgaa

SEQ ID NO: 85 - RNA, 14 nt, synthetic construct
  source 1..14: mol_type = other RNA; note = Xc1-Lk-Xc2 of Formula (I)
ttcatgaaaatgaa

SEQ ID NO: 86 - RNA, 10 nt, synthetic construct
  source 1..10: mol_type = other RNA; note = Xc1-Lk-Xc2 of Formula (I)
ttcgaaagaa

SEQ ID NO: 87 - RNA, 161 nt, synthetic construct
  source 1..161: mol_type = other RNA; note = Engineered tracrRNA for TnpB gRNA (MS1)
cttcactgataaagtggagaaccgcttcaccaaaagctgtcccttaggggattagaacttgagtgaaggtgggctgcttgcatcagcctaatgtcgagaagtgctttcttcggaaagtaaccctcgaaacaaattcagtgctcctctccaattctgcacaa

SEQ ID NO: 88 - RNA, 154 nt, synthetic construct
  source 1..154: mol_type = other RNA; note = Engineered tracrRNA for TnpB gRNA (MS1/MS3-1)
gataaagtggagaaccgcttcaccaaaagctgtcccttaggggattagaacttgagtgaaggtgggctgcttgcatcagcctaatgtcgagaagtgctttcttcggaaagtaaccctcgaaacaaattcagtgctcctctccaattctgcacaa

SEQ ID NO: 89 - RNA, 147 nt, synthetic construct
  source 1..147: mol_type = other RNA; note = Engineered tracrRNA for TnpB gRNA (MS1/MS3-2)
tggagaaccgcttcaccaaaagctgtcccttaggggattagaacttgagtgaaggtgggctgcttgcatcagcctaatgtcgagaagtgctttcttcggaaagtaaccctcgaaacaaattcagtgctcctctccaattctgcacaa

SEQ ID NO: 90 - RNA, 141 nt, synthetic construct
  source 1..141: mol_type = other RNA; note = Engineered tracrRNA for TnpB gRNA (MS1/MS3-3)
accgcttcaccaaaagctgtcccttaggggattagaacttgagtgaaggtgggctgcttgcatcagcctaatgtcgagaagtgctttcttcggaaagtaaccctcgaaacaaattcagtgctcctctccaattctgcacaa

SEQ ID NO: 91 - RNA, 154 nt, synthetic construct
  source 1..154: mol_type = other RNA; note = Engineered tracrRNA for TnpB gRNA (MS1/MS4*-1)
cttcactgataaagtggagaaccgcttcaccaaaagctgtcccttaggggattagaacttgagtgaaggtgggctgcttgcatcagcctaatgtcgagaagtgctttcttcggaaagtaaccctcgaaacaaattcagtgctcctctccaattc

SEQ ID NO: 92 - RNA, 148 nt, synthetic construct
  source 1..148: mol_type = other RNA; note = Engineered tracrRNA for TnpB gRNA (MS1/MS4*-2)
cttcactgataaagtggagaaccgcttcaccaaaagctgtcccttaggggattagaacttgagtgaaggtgggctgcttgcatcagcctaatgtcgagaagtgctttcttcggaaagtaaccctcgaaacaaattcagtgctcctctc

SEQ ID NO: 93 - RNA, 142 nt, synthetic construct
  source 1..142: mol_type = other RNA; note = Engineered tracrRNA for TnpB gRNA (MS1/MS4*-3)
cttcactgataaagtggagaaccgcttcaccaaaagctgtcccttaggggattagaacttgagtgaaggtgggctgcttgcatcagcctaatgtcgagaagtgctttcttcggaaagtaaccctcgaaacaaattcagtgct

SEQ ID NO: 94 - RNA, 155 nt, synthetic construct
  source 1..155: mol_type = other RNA; note = Engineered tracrRNA for TnpB gRNA (MS1/MS5-1)
cttcactgataaagtggagaaccgcttcaccaaaagctgtttagattagaacttgagtgaaggtgggctgcttgcatcagcctaatgtcgagaagtgctttcttcggaaagtaaccctcgaaacaaattcagtgctcctctccaattctgcacaa

SEQ ID NO: 95 - RNA, 148 nt, synthetic construct
  source 1..148: mol_type = other RNA; note = Engineered tracrRNA for TnpB gRNA (MS1/MS5-2)
cttcactgataaagtggagaaccgcttcaccaaaagcttaggaacttgagtgaaggtgggctgcttgcatcagcctaatgtcgagaagtgctttcttcggaaagtaaccctcgaaacaaattcagtgctcctctccaattctgcacaa

SEQ ID NO: 96 - RNA, 140 nt, synthetic construct
  source 1..140: mol_type = other RNA; note = Engineered tracrRNA for TnpB gRNA (MS1/MS5-3)
cttcactgataaagtggagaaccgcttcaccaattagttgagtgaaggtgggctgcttgcatcagcctaatgtcgagaagtgctttcttcggaaagtaaccctcgaaacaaattcagtgctcctctccaattctgcacaa

SEQ ID NO: 97 - RNA, 134 nt, synthetic construct
  source 1..134: mol_type = other RNA; note = Engineered tracrRNA for TnpB gRNA (MS1/MS3-3/MS4*-1)
accgcttcaccaaaagctgtcccttaggggattagaacttgagtgaaggtgggctgcttgcatcagcctaatgtcgagaagtgctttcttcggaaagtaaccctcgaaacaaattcagtgctcctctccaattc

SEQ ID NO: 98 - RNA, 128 nt, synthetic construct
  source 1..128: mol_type = other RNA; note = Engineered tracrRNA for TnpB gRNA (MS1/MS3-3/MS4*-2)
accgcttcaccaaaagctgtcccttaggggattagaacttgagtgaaggtgggctgcttgcatcagcctaatgtcgagaagtgctttcttcggaaagtaaccctcgaaacaaattcagtgctcctctc

SEQ ID NO: 99 - RNA, 122 nt, synthetic construct
  source 1..122: mol_type = other RNA; note = Engineered tracrRNA for TnpB gRNA (MS1/MS3-3/MS4*-3)
accgcttcaccaaaagctgtcccttaggggattagaacttgagtgaaggtgggctgcttgcatcagcctaatgtcgagaagtgctttcttcggaaagtaaccctcgaaacaaattcagtgct

SEQ ID NO: 100 - RNA, 142 nt, synthetic construct
  source 1..142: mol_type = other RNA; note = Engineered tracrRNA for TnpB gRNA (MS1/MS4*-2/MS5-1)
cttcactgataaagtggagaaccgcttcaccaaaagctgtttagattagaacttgagtgaaggtgggctgcttgcatcagcctaatgtcgagaagtgctttcttcggaaagtaaccctcgaaacaaattcagtgctcctctc

SEQ ID NO: 101 - RNA, 135 nt, synthetic construct
  source 1..135: mol_type = other RNA; note = Engineered tracrRNA for TnpB gRNA (MS1/MS4*-2/MS5-2)
cttcactgataaagtggagaaccgcttcaccaaaagcttaggaacttgagtgaaggtgggctgcttgcatcagcctaatgtcgagaagtgctttcttcggaaagtaaccctcgaaacaaattcagtgctcctctc

SEQ ID NO: 102 - RNA, 127 nt, synthetic construct
  source 1..127: mol_type = other RNA; note = Engineered tracrRNA for TnpB gRNA (MS1/MS4*-2/MS5-3)
cttcactgataaagtggagaaccgcttcaccaattagttgagtgaaggtgggctgcttgcatcagcctaatgtcgagaagtgctttcttcggaaagtaaccctcgaaacaaattcagtgctcctctc

SEQ ID NO: 103 - RNA, 135 nt, synthetic construct
  source 1..135: mol_type = other RNA; note = Engineered tracrRNA for TnpB gRNA (MS1/MS3-3/MS5-1)
accgcttcaccaaaagctgtttagattagaacttgagtgaaggtgggctgcttgcatcagcctaatgtcgagaagtgctttcttcggaaagtaaccctcgaaacaaattcagtgctcctctccaattctgcacaa

SEQ ID NO: 104 - RNA, 128 nt, synthetic construct
  source 1..128: mol_type = other RNA; note = Engineered tracrRNA for TnpB gRNA (MS1/MS3-3/MS5-2)
accgcttcaccaaaagcttaggaacttgagtgaaggtgggctgcttgcatcagcctaatgtcgagaagtgctttcttcggaaagtaaccctcgaaacaaattcagtgctcctctccaattctgcacaa

SEQ ID NO: 105 - RNA, 120 nt, synthetic construct
  source 1..120: mol_type = other RNA; note = Engineered tracrRNA for TnpB gRNA (MS1/MS3-3/MS5-3)
accgcttcaccaattagttgagtgaaggtgggctgcttgcatcagcctaatgtcgagaagtgctttcttcggaaagtaaccctcgaaacaaattcagtgctcctctccaattctgcacaa

SEQ ID NO: 106 - RNA, 107 nt, synthetic construct
  source 1..107: mol_type = other RNA; note = Engineered tracrRNA for TnpB gRNA (MS1/MS3-3/MS4*-2/MS5-3)
accgcttcaccaattagttgagtgaaggtgggctgcttgcatcagcctaatgtcgagaagtgctttcttcggaaagtaaccctcgaaacaaattcagtgctcctctc

SEQ ID NO: 107 - RNA, 140 nt, synthetic construct
  source 1..140: mol_type = other RNA; note = Engineered tracrRNA for TnpB gRNA (MF)
cttcactgataaagtggagaaccgcttcaccaaaagctgtcccttaggggattagaacttgagtgaaggtgggctgcttgcatcagcctaatgtcgagaagtgctttcttcggaaagtaaccctcgaaacaaattcattt

SEQ ID NO: 108 - RNA, 133 nt, synthetic construct
  source 1..133: mol_type = other RNA; note = Engineered tracrRNA for TnpB gRNA (MF/MS3-1)
gataaagtggagaaccgcttcaccaaaagctgtcccttaggggattagaacttgagtgaaggtgggctgcttgcatcagcctaatgtcgagaagtgctttcttcggaaagtaaccctcgaaacaaattcattt

SEQ ID NO: 109 - RNA, 126 nt, synthetic construct
  source 1..126: mol_type = other RNA; note = Engineered tracrRNA for TnpB gRNA (MF/MS3-2)
tggagaaccgcttcaccaaaagctgtcccttaggggattagaacttgagtgaaggtgggctgcttgcatcagcctaatgtcgagaagtgctttcttcggaaagtaaccctcgaaacaaattcattt

SEQ ID NO: 110 - RNA, 120 nt, synthetic construct
  source 1..120: mol_type = other RNA; note = Engineered tracrRNA for TnpB gRNA (MF/MS3-3)
accgcttcaccaaaagctgtcccttaggggattagaacttgagtgaaggtgggctgcttgcatcagcctaatgtcgagaagtgctttcttcggaaagtaaccctcgaaacaaattcattt

SEQ ID NO: 111 - RNA, 138 nt, synthetic construct
  source 1..138: mol_type = other RNA; note = Engineered tracrRNA for TnpB gRNA (MF/MS4-1)
cttcactgataaagtggagaaccgcttcaccaaaagctgtcccttaggggattagaacttgagtgaaggtgggctgcttgcatcagcctaatgtcgagaagtgctttcttcggaaagtaaccctcgaaacaaattcat

SEQ ID NO: 112 - RNA, 136 nt, synthetic construct
  source 1..136: mol_type = other RNA; note = Engineered tracrRNA for TnpB gRNA (MF/MS4-2)
cttcactgataaagtggagaaccgcttcaccaaaagctgtcccttaggggattagaacttgagtgaaggtgggctgcttgcatcagcctaatgtcgagaagtgctttcttcggaaagtaaccctcgaaacaaattc

SEQ ID NO: 113 - RNA, 133 nt, synthetic construct
  source 1..133: mol_type = other RNA; note = Engineered tracrRNA for TnpB gRNA (MF/MS4-3)
cttcactgataaagtggagaaccgcttcaccaaaagctgtcccttaggggattagaacttgagtgaaggtgggctgcttgcatcagcctaatgtcgagaagtgctttcttcggaaagtaaccctcgaaacaaa

SEQ ID NO: 114 - RNA, 134 nt, synthetic construct
  source 1..134: mol_type = other RNA; note = Engineered tracrRNA for TnpB gRNA (MF/MS5-1)
cttcactgataaagtggagaaccgcttcaccaaaagctgtttagattagaacttgagtgaaggtgggctgcttgcatcagcctaatgtcgagaagtgctttcttcggaaagtaaccctcgaaacaaattcattt

SEQ ID NO: 115 - RNA, 129 nt, synthetic construct
  source 1..129: mol_type = other RNA; note = Engineered tracrRNA for TnpB gRNA (MF/MS5-2)
cttcactgataaagtggagaaccgcttcaccaaaagctttagagaacttgagtgaaggtgggctgcttgcatcagcctaatgtcgagaagtgctttcttcggaaagtaaccctcgaaacaaattcattt

SEQ ID NO: 116 - RNA, 119 nt, synthetic construct
  source 1..119: mol_type = other RNA; note = Engineered tracrRNA for TnpB gRNA (MF/MS5-3)
cttcactgataaagtggagaaccgcttcaccaattagttgagtgaaggtgggctgcttgcatcagcctaatgtcgagaagtgctttcttcggaaagtaaccctcgaaacaaattcattt

SEQ ID NO: 117 - RNA, 113 nt, synthetic construct
  source 1..113: mol_type = other RNA; note = Engineered tracrRNA for TnpB gRNA (MF/MS5)
cttcactgataaagtggagaaccgcttcacttagagtgaaggtgggctgcttgcatcagcctaatgtcgagaagtgctttcttcggaaagtaaccctcgaaacaaattcattt

SEQ ID NO: 118 - RNA, 118 nt, synthetic construct
  source 1..118: mol_type = other RNA; note = Engineered tracrRNA for TnpB gRNA (MF/MS3-3/MS4-1)
accgcttcaccaaaagctgtcccttaggggattagaacttgagtgaaggtgggctgcttgcatcagcctaatgtcgagaagtgctttcttcggaaagtaaccctcgaaacaaattcat

SEQ ID NO: 119 - RNA, 116 nt, synthetic construct
  source 1..116: mol_type = other RNA; note = Engineered tracrRNA for TnpB gRNA (MF/MS3-3/MS4-2)
accgcttcaccaaaagctgtcccttaggggattagaacttgagtgaaggtgggctgcttgcatcagcctaatgtcgagaagtgctttcttcggaaagtaaccctcgaaacaaattc

SEQ ID NO: 120 - RNA, 113 nt, synthetic construct
  source 1..113: mol_type = other RNA; note = Engineered tracrRNA for TnpB gRNA (MF/MS3-3/MS4-3)
accgcttcaccaaaagctgtcccttaggggattagaacttgagtgaaggtgggctgcttgcatcagcctaatgtcgagaagtgctttcttcggaaagtaaccctcgaaacaaa

SEQ ID NO: 121 - RNA, 127 nt, synthetic construct
  source 1..127: mol_type = other RNA; note = Engineered tracrRNA for TnpB gRNA (MF/MS4-3/MS5-1)
cttcactgataaagtggagaaccgcttcaccaaaagctgtttagattagaacttgagtgaaggtgggctgcttgcatcagcctaatgtcgagaagtgctttcttcggaaagtaaccctcgaaacaaa

SEQ ID NO: 122 - RNA, 122 nt, synthetic construct
  source 1..122: mol_type = other RNA; note = Engineered tracrRNA for TnpB gRNA (MF/MS4-3/MS5-2)
cttcactgataaagtggagaaccgcttcaccaaaagctttagagaacttgagtgaaggtgggctgcttgcatcagcctaatgtcgagaagtgctttcttcggaaagtaaccctcgaaacaaa

SEQ ID NO: 123 - RNA, 112 nt, synthetic construct
  source 1..112: mol_type = other RNA; note = Engineered tracrRNA for TnpB gRNA (MF/MS4-3/MS5-3)
cttcactgataaagtggagaaccgcttcaccaattagttgagtgaaggtgggctgcttgcatcagcctaatgtcgagaagtgctttcttcggaaagtaaccctcgaaacaaa

SEQ ID NO: 124 - RNA, 106 nt, synthetic construct
  source 1..106: mol_type = other RNA; note = Engineered tracrRNA for TnpB gRNA (MF/MS4-3/MS5)
cttcactgataaagtggagaaccgcttcacttagagtgaaggtgggctgcttgcatcagcctaatgtcgagaagtgctttcttcggaaagtaaccctcgaaacaaa

SEQ ID NO: 125 - RNA, 114 nt, synthetic construct
  source 1..114: mol_type = other RNA; note = Engineered tracrRNA for TnpB gRNA (MF/MS3-3/MS5-1)
accgcttcaccaaaagctgtttagattagaacttgagtgaaggtgggctgcttgcatcagcctaatgtcgagaagtgctttcttcggaaagtaaccctcgaaacaaattcattt

SEQ ID NO: 126 - RNA, 109 nt, synthetic construct
  source 1..109: mol_type = other RNA; note = Engineered tracrRNA for TnpB gRNA (MF/MS3-3/MS5-2)
accgcttcaccaaaagctttagagaacttgagtgaaggtgggctgcttgcatcagcctaatgtcgagaagtgctttcttcggaaagtaaccctcgaaacaaattcattt

SEQ ID NO: 127 - RNA, 99 nt, synthetic construct
  source 1..99: mol_type = other RNA; note = Engineered tracrRNA for TnpB gRNA (MF/MS3-3/MS5-3)
accgcttcaccaattagttgagtgaaggtgggctgcttgcatcagcctaatgtcgagaagtgctttcttcggaaagtaaccctcgaaacaaattcattt

SEQ ID NO: 128 - RNA, 93 nt, synthetic construct
  source 1..93: mol_type = other RNA; note = Engineered tracrRNA for TnpB gRNA (MF/MS3-3/MS5)
accgcttcacttagagtgaaggtgggctgcttgcatcagcctaatgtcgagaagtgctttcttcggaaagtaaccctcgaaacaaattcattt

SEQ ID NO: 129 - RNA, 92 nt, synthetic construct
  source 1..92: mol_type = other RNA; note = Engineered tracrRNA for TnpB gRNA (MF/MS3-3/MS4-3/MS5-3)
accgcttcaccaattagttgagtgaaggtgggctgcttgcatcagcctaatgtcgagaagtgctttcttcggaaagtaaccctcgaaacaaa

SEQ ID NO: 130 - RNA, 91 nt, synthetic construct
  source 1..91: mol_type = other RNA; note = Engineered tracrRNA for TnpB gRNA (MF/MS3-3/MS4-1/MS5)
accgcttcacttagagtgaaggtgggctgcttgcatcagcctaatgtcgagaagtgctttcttcggaaagtaaccctcgaaacaaattcat

SEQ ID NO: 131 - RNA, 89 nt, synthetic construct
  source 1..89: mol_type = other RNA; note = Engineered tracrRNA for TnpB gRNA (MF/MS3-3/MS4-2/MS5)
accgcttcacttagagtgaaggtgggctgcttgcatcagcctaatgtcgagaagtgctttcttcggaaagtaaccctcgaaacaaattc

SEQ ID NO: 132 - RNA, 86 nt, synthetic construct
  source 1..86: mol_type = other RNA; note = Engineered tracrRNA for TnpB gRNA (MF/MS3-3/MS4-3/MS5)
accgcttcacttagagtgaaggtgggctgcttgcatcagcctaatgtcgagaagtgctttcttcggaaagtaaccctcgaaacaaa

SEQ ID NO: 133 - RNA, 37 nt, synthetic construct
  source 1..37: mol_type = other RNA; note = Engineered crRNA for TnpB gRNA (MS1)
gttgcagaacccgaatagagcaatgaaggaatgcaac

SEQ ID NO: 134 - RNA, 31 nt, synthetic construct
  source 1..31: mol_type = other RNA; note = Engineered crRNA for TnpB gRNA (MS1/MS4*-1)
gaacccgaatagagcaatgaaggaatgcaac

SEQ ID NO: 135 - RNA, 25 nt, synthetic construct
  source 1..25: mol_type = other RNA; note = Engineered crRNA for TnpB gRNA (MS1/MS4*-2)
gaatagagcaatgaaggaatgcaac

SEQ ID NO: 136 - RNA, 19 nt, synthetic construct
  source 1..19: mol_type = other RNA; note = Engineered crRNA for TnpB gRNA (MS1/MS4*-3)
agcaatgaaggaatgcaac

SEQ ID NO: 137 - RNA, 17 nt, synthetic construct
  source 1..17: mol_type = other RNA; note = Engineered crRNA for TnpB gRNA (MF)
gaatgaaggaatgcaac

SEQ ID NO: 138 - RNA, 15 nt, synthetic construct
  source 1..15: mol_type = other RNA; note = Engineered crRNA for TnpB gRNA (MF/MS4-1)
atgaaggaatgcaac

SEQ ID NO: 139 - RNA, 13 nt, synthetic construct
  source 1..13: mol_type = other RNA; note = Engineered crRNA for TnpB gRNA (MF/MS4-2)
gaaggaatgcaac

SEQ ID NO: 140 - RNA, 10 nt, synthetic construct
  source 1..10: mol_type = other RNA; note = Engineered crRNA for TnpB gRNA (MF/MS4-3)
ggaatgcaac

SEQ ID NO: 141 - RNA, 68 nt, synthetic construct
  source 1..68: mol_type = other RNA; note = Engineered crRNA for TnpB gRNA (MS1/MS2)
  misc_feature 38..57: note = n is a, c, g or u
gttgcagaacccgaatagagcaatgaaggaatgcaacnnnnnnnnnnnnnnnnnnnnttttatttttt

SEQ ID NO: 142 - RNA, 62 nt, synthetic construct
  source 1..62: mol_type = other RNA; note = Engineered crRNA for TnpB gRNA (MS1/MS2/MS4*-1)
  misc_feature 32..51: note = n is a, c, g or u
gaacccgaatagagcaatgaaggaatgcaacnnnnnnnnnnnnnnnnnnnnttttatttttt

SEQ ID NO: 143 - RNA, 56 nt, synthetic construct
  source 1..56: mol_type = other RNA; note = Engineered crRNA for TnpB gRNA (MS1/MS2/MS4*-2)
  misc_feature 26..45: note = n is a, c, g or u
gaatagagcaatgaaggaatgcaacnnnnnnnnnnnnnnnnnnnnttttatttttt

SEQ ID NO: 144 - RNA, 50 nt, synthetic construct
  source 1..50: mol_type = other RNA; note = Engineered crRNA for TnpB gRNA (MS1/MS2/MS4*-3)
  misc_feature 20..39: note = n is a, c, g or u
agcaatgaaggaatgcaacnnnnnnnnnnnnnnnnnnnnttttatttttt

SEQ ID NO: 145 - RNA, 48 nt, synthetic construct
  source 1..48: mol_type = other RNA; note = Engineered crRNA for TnpB gRNA (MF/MS2)
  misc_feature 18..37: note = n is a, c, g or u
gaatgaaggaatgcaacnnnnnnnnnnnnnnnnnnnnttttatttttt

SEQ ID NO: 146 - RNA, 46 nt, synthetic construct
  source 1..46: mol_type = other RNA; note = Engineered crRNA for TnpB gRNA (MF/MS2/MS4-1)
  misc_feature 16..35: note = n is a, c, g or u
atgaaggaatgcaacnnnnnnnnnnnnnnnnnnnnttttatttttt

SEQ ID NO: 147 - RNA, 44 nt, synthetic construct
  source 1..44: mol_type = other RNA; note = Engineered crRNA for TnpB gRNA (MF/MS2/MS4-2)
  misc_feature 14..33: note = n is a, c, g or u
gaaggaatgcaacnnnnnnnnnnnnnnnnnnnnttttatttttt

SEQ ID NO: 148 - RNA, 41 nt, synthetic construct
  source 1..41: mol_type = other RNA; note = Engineered crRNA for TnpB gRNA (MF/MS2/MS4-3)
  misc_feature 11..30: note = n is a, c, g or u
ggaatgcaacnnnnnnnnnnnnnnnnnnnnttttatttttt

SEQ ID NO: 149 - RNA, 222 nt, synthetic construct
  source 1..222: mol_type = other RNA; note = Engineered sgRNA with modification of MS1 for TnpB
  misc_feature 203..222: note = n is a, c, g or u
cttcactgataaagtggagaaccgcttcaccaaaagctgtcccttaggggattagaacttgagtgaaggtgggctgcttgcatcagcctaatgtcgagaagtgctttcttcggaaagtaaccctcgaaacaaattcagtgctcctctccaattctgcacaagaaagttgcagaacccgaatagagcaatgaaggaatgcaacnnnnnnnnnnnnnnnnnnnn

SEQ ID NO: 150 - RNA, 233 nt, synthetic construct
  source 1..233: mol_type = other RNA; note = Engineered sgRNA with modification of MS1/MS2 for TnpB
  misc_feature 203..222: note = n is a, c, g or u
cttcactgataaagtggagaaccgcttcaccaaaagctgtcccttaggggattagaacttgagtgaaggtgggctgcttgcatcagcctaatgtcgagaagtgctttcttcggaaagtaaccctcgaaacaaattcagtgctcctctccaattctgcacaagaaagttgcagaacccgaatagagcaatgaaggaatgcaacnnnnnnnnnnnnnnnnnnnnttttatttttt

SEQ ID NO: 151 - RNA, 213 nt, synthetic construct
  source 1..213: mol_type = other RNA; note = Engineered sgRNA with modification of MS1/MS2/MS3 for TnpB
  misc_structure 183..202: note = n is a, c, g or u
accgcttcaccaaaagctgtcccttaggggattagaacttgagtgaaggtgggctgcttgcatcagcctaatgtcgagaagtgctttcttcggaaagtaaccctcgaaacaaattcagtgctcctctccaattctgcacaagaaagttgcagaacccgaatagagcaatgaaggaatgcaacnnnnnnnnnnnnnnnnnnnnttttatttttt

SEQ ID NO: 152 - RNA, 158 nt, synthetic construct
  source 1..158: mol_type = other RNA; note = Engineered sgRNA with modification of MS2/MS3/MS4 for TnpB
  misc_feature 128..147: note = n is a, c, g or u
accgcttcaccaaaagctgtcccttaggggattagaacttgagtgaaggtgggctgcttgcatcagcctaatgtcgagaagtgctttcttcggaaagtaaccctcgaaacaaagaaaggaatgcaacnnnnnnnnnnnnnnnnnnnnttttatttttt

SEQ ID NO: 153 - RNA, 131 nt, synthetic construct
  source 1..131: mol_type = other RNA; note = Engineered sgRNA with modification of MS2/MS3/MS4/MS5 for TnpB
  misc_feature 99..118: note = n is a, c, g or u
accgcttcacttagagtgaaggtgggctgcttgcatcagcctaatgtcgagaagtgctttcttcggaaagtaaccctcgaaacaaagaaaggaatgcaacnnnnnnnnnnnnnnnnnnnnttttatttttt

SEQ ID NO: 154 - RNA, 215 nt, synthetic construct
  source 1..215: mol_type = other RNA; note = Engineered sgRNA with modification of MS1/MS3-1 for TnpB
  misc_feature 196..215: note = n is a, c, g or u
gataaagtggagaaccgcttcaccaaaagctgtcccttaggggattagaacttgagtgaaggtgggctgcttgcatcagcctaatgtcgagaagtgctttcttcggaaagtaaccctcgaaacaaattcagtgctcctctccaattctgcacaagaaagttgcagaacccgaatagagcaatgaaggaatgcaacnnnnnnnnnnnnnnnnnnnn

SEQ ID NO: 155 - RNA, 208 nt, synthetic construct
  source 1..208: mol_type = other RNA; note = Engineered sgRNA with modification of MS1/MS3-2 for TnpB
  misc_feature 189..208: note = n is a, c, g or u
tggagaaccgcttcaccaaaagctgtcccttaggggattagaacttgagtgaaggtgggctgcttgcatcagcctaatgtcgagaagtgctttcttcggaaagtaaccctcgaaacaaattcagtgctcctctccaattctgcacaagaaagttgcagaacccgaatagagcaatgaaggaatgcaacnnnnnnnnnnnnnnnnnnnn

SEQ ID NO: 156 - RNA, 202 nt, synthetic construct
  source 1..202: mol_type = other RNA; note = Engineered sgRNA with modification of MS1/MS3-3 for TnpB
  misc_feature 183..202: note = n is a, c, g or u
accgcttcaccaaaagctgtcccttaggggattagaacttgagtgaaggtgggctgcttgcatcagcctaatgtcgagaagtgctttcttcggaaagtaaccctcgaaacaaattcagtgctcctctccaattctgcacaagaaagttgcagaacccgaatagagcaatgaaggaatgcaacnnnnnnnnnnnnnnnnnnnn

SEQ ID NO: 157 - RNA, 209 nt, synthetic construct
  source 1..209: mol_type = other RNA; note = Engineered sgRNA with modification of MS1/MS4*-1 for TnpB
  misc_feature 190..209: note = n is a, c, g or u
cttcactgataaagtggagaaccgcttcaccaaaagctgtcccttaggggattagaacttgagtgaaggtgggctgcttgcatcagcctaatgtcgagaagtgctttcttcggaaagtaaccctcgaaacaaattcagtgctcctctccaattcgaaagaacccgaatagagcaatgaaggaatgcaacnnnnnnnnnnnnnnnnnnnn

SEQ ID NO: 158 - RNA, 197 nt, synthetic construct
  source 1..197: mol_type = other RNA; note = Engineered sgRNA with modification of MS1/MS4*-2 for TnpB
  misc_feature 178..197: note = n is a, c, g or u
cttcactgataaagtggagaaccgcttcaccaaaagctgtcccttaggggattagaacttgagtgaaggtgggctgcttgcatcagcctaatgtcgagaagtgctttcttcggaaagtaaccctcgaaacaaattcagtgctcctctcgaaagaatagagcaatgaaggaatgcaacnnnnnnnnnnnnnnnnnnnn

SEQ ID NO: 159 - RNA, 185 nt, synthetic construct
  source 1..185: mol_type = other RNA; note = Engineered sgRNA with modification of MS1/MS4*-3 for TnpB
  misc_feature 166..185: note = n is a, c, g or u
cttcactgataaagtggagaaccgcttcaccaaaagctgtcccttaggggattagaacttgagtgaaggtgggctgcttgcatcagcctaatgtcgagaagtgctttcttcggaaagtaaccctcgaaacaaattcagtgctgaaaagcaatgaaggaatgcaacnnnnnnnnnnnnnnnnnnnn

SEQ ID NO: 160 - RNA, 216 nt, synthetic construct
  source 1..216: mol_type = other RNA; note = Engineered sgRNA with modification of MS1/MS5-1 for TnpB
  misc_feature 197..216: note = n is a, c, g or u
cttcactgataaagtggagaaccgcttcaccaaaagctgtttagattagaacttgagtgaaggtgggctgcttgcatcagcctaatgtcgagaagtgctttcttcggaaagtaaccctcgaaacaaattcagtgctcctctccaattctgcacaagaaagttgcagaacccgaatagagcaatgaaggaatgcaacnnnnnnnnnnnnnnnnnnnn

SEQ ID NO: 161 - RNA, 209 nt, synthetic construct
  source 1..209: mol_type = other RNA; note = Engineered sgRNA with modification of MS1/MS5-2 for TnpB
  misc_feature 190..209: note = n is a, c, g or u
cttcactgataaagtggagaaccgcttcaccaaaagcttaggaacttgagtgaaggtgggctgcttgcatcagcctaatgtcgagaagtgctttcttcggaaagtaaccctcgaaacaaattcagtgctcctctccaattctgcacaagaaagttgcagaacccgaatagagcaatgaaggaatgcaacnnnnnnnnnnnnnnnnnnnn

SEQ ID NO: 162 - RNA, 201 nt, synthetic construct
  source 1..201: mol_type = other RNA; note = Engineered sgRNA with modification of MS1/MS5-3 for TnpB
  misc_feature 182..201: note = n is a, c, g or u
cttcactgataaagtggagaaccgcttcaccaattagttgagtgaaggtgggctgcttgcatcagcctaatgtcgagaagtgctttcttcggaaagtaaccctcgaaacaaattcagtgctcctctccaattctgcacaagaaagttgcagaacccgaatagagcaatgaaggaatgcaacnnnnnnnnnnnnnnnnnnnn

SEQ ID NO: 163 - RNA, 206 nt, synthetic construct
  source 1..206: mol_type = other RNA; note = Engineered sgRNA with modification of MS1/MS2/MS4*-2 for TnpB
  misc_feature 178..197: note = n is a, c, g or u
cttcactgataaagtggagaaccgcttcaccaaaagctgtcccttaggggattagaacttgagtgaaggtgggctgcttgcatcagcctaatgtcgagaagtgctttcttcggaaagtaaccctcgaaacaaattcagtgctcctctcgaaagaatagagcaatgaaggaatgcaacnnnnnnnnnnnnnnnnnnnnttttatttt

SEQ ID NO: 164 - RNA, 177 nt, synthetic construct
  source 1..177: mol_type = other RNA
accgcttcaccaaaagctgtcccttaggggattagaacttgagtgaaggtgggctgcttgcatcagcctaatgtcgagaagtgctttcttcggaaagtaaccctcgaaacaaattcagtgctcctctcgaaagaatagagcaatgaaggaatgcaacnnnnnnnnnnnnnnnnnnnn

SEQ ID NO: 165 - RNA, 210 nt, synthetic construct
  source 1..210: mol_type = other RNA; note = Engineered sgRNA with modification of MS1/MS2/MS5-3 for TnpB
  misc_feature 182..201: note = n is a, c, g or u
cttcactgataaagtggagaaccgcttcaccaattagttgagtgaaggtgggctgcttgcatcagcctaatgtcgagaagtgctttcttcggaaagtaaccctcgaaacaaattcagtgctcctctccaattctgcacaagaaagttgcagaacccgaatagagcaatgaaggaatgcaacnnnnnnnnnnnnnnnnnnnnttttatttt

SEQ ID NO: 166 - RNA, 181 nt, synthetic construct
  source 1..181: mol_type = other RNA; note = Engineered sgRNA with modification of MS1/MS3-3/MS5-3 for TnpB
  misc_feature 162..181: note = n is a, c, g or u
accgcttcaccaattagttgagtgaaggtgggctgcttgcatcagcctaatgtcgagaagtgctttcttcggaaagtaaccctcgaaacaaattcagtgctcctctccaattctgcacaagaaagttgcagaacccgaatagagcaatgaaggaatgcaacnnnnnnnnnnnnnnnnnnnn

SEQ ID NO: 167 - RNA, 176 nt, synthetic construct
  source 1..176: mol_type = other RNA; note = Engineered sgRNA with modification of MS1/MS4*-2/MS5-3 for TnpB
  misc_feature 157..176: note = n is a, c, g or u
cttcactgataaagtggagaaccgcttcaccaattagttgagtgaaggtgggctgcttgcatcagcctaatgtcgagaagtgctttcttcggaaagtaaccctcgaaacaaattcagtgctcctctcgaaagaatagagcaatgaaggaatgcaacnnnnnnnnnnnnnnnnnnnn

SEQ ID NO: 168 - RNA, 186 nt, synthetic construct
  source 1..186: mol_type = other RNA; note = Engineered sgRNA with modification of MS1/MS2/MS3-3/MS4*-2 for TnpB
  misc_feature 158..177: note = n is a, c, g or u
accgcttcaccaaaagctgtcccttaggggattagaacttgagtgaaggtgggctgcttgcatcagcctaatgtcgagaagtgctttcttcggaaagtaaccctcgaaacaaattcagtgctcctctcgaaagaatagagcaatgaaggaatgcaacnnnnnnnnnnnnnnnnnnnnttttatttt

SEQ ID NO: 169 - RNA, 190 nt, synthetic construct
  source 1..190: mol_type = other RNA; note = Engineered sgRNA with modification of MS1/MS2/MS3-3/MS5-3 for TnpB
  misc_feature 162..181: note = n is a, c, g or u
accgcttcaccaattagttgagtgaaggtgggctgcttgcatcagcctaatgtcgagaagtgctttcttcggaaagtaaccctcgaaacaaattcagtgctcctctccaattctgcacaagaaagttgcagaacccgaatagagcaatgaaggaatgcaacnnnnnnnnnnnnnnnnnnnnttttatttt

SEQ ID NO: 170 - RNA, 185 nt, synthetic construct
  source 1..185: mol_type = other RNA; note = Engineered sgRNA with modification of MS1/MS2/MS4*-2/MS5-3 for TnpB
  misc_feature 157..176: note = n is a, c, g or u
cttcactgataaagtggagaaccgcttcaccaattagttgagtgaaggtgggctgcttgcatcagcctaatgtcgagaagtgctttcttcggaaagtaaccctcgaaacaaattcagtgctcctctcgaaagaatagagcaatgaaggaatgcaacnnnnnnnnnnnnnnnnnnnnttttatttt

SEQ ID NO: 171 - RNA, 156 nt, synthetic construct
  source 1..156: mol_type = other RNA; note = Engineered sgRNA with modification of MS1/MS3-3/MS4*-2/MS5-3 for TnpB
  misc_feature 137..156: note = n is a, c, g or u
accgcttcaccaattagttgagtgaaggtgggctgcttgcatcagcctaatgtcgagaagtgctttcttcggaaagtaaccctcgaaacaaattcagtgctcctctcgaaagaatagagcaatgaaggaatgcaacnnnnnnnnnnnnnnnnnnnn

SEQ ID NO: 172 - RNA, 165 nt, synthetic construct
  source 1..165: mol_type = other RNA; note = Engineered sgRNA with modification of MS1/MS2/MS3-3/MS4*-2/MS5-3 for TnpB
  misc_feature 137..156: note = n is a, c, g or u
accgcttcaccaattagttgagtgaaggtgggctgcttgcatcagcctaatgtcgagaagtgctttcttcggaaagtaaccctcgaaacaaattcagtgctcctctcgaaagaatagagcaatgaaggaatgcaacnnnnnnnnnnnnnnnnnnnnttttatttt

SEQ ID NO: 173 - RNA, 181 nt, synthetic construct
  source 1..181: mol_type = other RNA; note = Mature form sgRNA for TnpB
  misc_feature 162..181: note = n is a, c, g or u
cttcactgataaagtggagaaccgcttcaccaaaagctgtcccttaggggattagaacttgagtgaaggtgggctgcttgcatcagcctaatgtcgagaagtgctttcttcggaaagtaaccctcgaaacaaattcatttgaaagaatgaaggaatgcaacnnnnnnnnnnnnnnnnnnnn

SEQ ID NO: 174 - RNA, 174 nt, synthetic construct
  source 1..174: mol_type = other RNA; note = Mature form sgRNA with modification of MS3-1 for TnpB
  misc_feature 155..174: note = n is a, c, g or u
gataaagtggagaaccgcttcaccaaaagctgtcccttaggggattagaacttgagtgaaggtgggctgcttgcatcagcctaatgtcgagaagtgctttcttcggaaagtaaccctcgaaacaaattcatttgaaagaatgaaggaatgcaacnnnnnnnnnnnnnnnnnnnn

SEQ ID NO: 175 - RNA, 167 nt, synthetic construct
  source 1..167: mol_type = other RNA; note = Mature form sgRNA with modification of MS3-2 for TnpB
  misc_feature 148..167: note = n is a, c, g or u
tggagaaccgcttcaccaaaagctgtcccttaggggattagaacttgagtgaaggtgggctgcttgcatcagcctaatgtcgagaagtgctttcttcggaaagtaaccctcgaaacaaattcatttgaaagaatgaaggaatgcaacnnnnnnnnnnnnnnnnnnnn

SEQ ID NO: 176 - RNA, 161 nt, synthetic construct
  source 1..161: mol_type = other RNA; note = Mature form sgRNA with modification of MS3-3 for TnpB
  misc_feature 142..161: note = n is a, c, g or u
accgcttcaccaaaagctgtcccttaggggattagaacttgagtgaaggtgggctgcttgcatcagcctaatgtcgagaagtgctttcttcggaaagtaaccctcgaaacaaattcatttgaaagaatgaaggaatgcaacnnnnnnnnnnnnnnnnnnnn

SEQ ID NO: 177 - RNA, 177 nt, synthetic construct
  source 1..177: mol_type = other RNA; note = Mature form sgRNA with modification of MS4-1 for TnpB
  misc_feature 158..177: note = n is a, c, g or u
cttcactgataaagtggagaaccgcttcaccaaaagctgtcccttaggggattagaacttgagtgaaggtgggctgcttgcatcagcctaatgtcgagaagtgctttcttcggaaagtaaccctcgaaacaaattcatgaaaatgaaggaatgcaacnnnnnnnnnnnnnnnnnnnn

SEQ ID NO: 178 - RNA, 173 nt, synthetic construct
  source 1..173: mol_type = other RNA; note = Mature form sgRNA with modification of MS4-2 for TnpB
  misc_feature 154..173: note = n is a, c, g or u
cttcactgataaagtggagaaccgcttcaccaaaagctgtcccttaggggattagaacttgagtgaaggtgggctgcttgcatcagcctaatgtcgagaagtgctttcttcggaaagtaaccctcgaaacaaattcgaaagaaggaatgcaacnnnnnnnnnnnnnnnnnnnn

SEQ ID NO: 179 - RNA, 167 nt, synthetic construct
  source 1..167: mol_type = other RNA; note = Mature form sgRNA with modification of MS4-3 for TnpB
  misc_feature 148..167: note = n is a, c, g or u
cttcactgataaagtggagaaccgcttcaccaaaagctgtcccttaggggattagaacttgagtgaaggtgggctgcttgcatcagcctaatgtcgagaagtgctttcttcggaaagtaaccctcgaaacaaagaaaggaatgcaacnnnnnnnnnnnnnnnnnnnn

SEQ ID NO: 180 - RNA, 175 nt, synthetic construct
  source 1..175: mol_type = other RNA; note = Mature form sgRNA with modification of MS5-1 for TnpB
  misc_feature 156..175: note = n is a, c, g or u
cttcactgataaagtggagaaccgcttcaccaaaagctgtttagattagaacttgagtgaaggtgggctgcttgcatcagcctaatgtcgagaagtgctttcttcggaaagtaaccctcgaaacaaattcatttgaaagaatgaaggaatgcaacnnnnnnnnnnnnnnnnnnnn

SEQ ID NO: 181 - RNA, 170 nt, synthetic construct
  source 1..170: mol_type = other RNA; note = Mature form sgRNA with modification of MS5-2 for TnpB
  misc_feature 151..170: note = n is a, c, g or u
cttcactgataaagtggagaaccgcttcaccaaaagctttagagaacttgagtgaaggtgggctgcttgcatcagcctaatgtcgagaagtgctttcttcggaaagtaaccctcgaaacaaattcatttgaaagaatgaaggaatgcaacnnnnnnnnnnnnnnnnnnnn

SEQ ID NO: 182 - RNA, 160 nt, synthetic construct
  source 1..160: mol_type = other RNA; note = Mature form sgRNA with modification of MS5-3 for TnpB
  misc_feature 141..160: note = n is a, c, g or u
cttcactgataaagtggagaaccgcttcaccaattagttgagtgaaggtgggctgcttgcatcagcctaatgtcgagaagtgctttcttcggaaagtaaccctcgaaacaaattcatttgaaagaatgaaggaatgcaacnnnnnnnnnnnnnnnnnnnn

SEQ ID NO: 183 - RNA, 147 nt, synthetic construct
  source 1..147: mol_type = other RNA; note = Mature form sgRNA with modification of MS3-3/MS4-3 for TnpB
  misc_feature 128..147: note = n is a, c, g or u
accgcttcaccaaaagctgtcccttaggggattagaacttgagtgaaggtgggctgcttgcatcagcctaatgtcgagaagtgctttcttcggaaagtaaccctcgaaacaaagaaaggaatgcaacnnnnnnnnnnnnnnnnnnnn

SEQ ID NO: 184 - RNA, 140 nt, synthetic construct
  source 1..140: mol_type = other RNA; note = Mature form sgRNA with modification of MS3-3/MS5-3 for TnpB
  misc_feature 121..140: note = n is a, c, g or u
accgcttcaccaattagttgagtgaaggtgggctgcttgcatcagcctaatgtcgagaagtgctttcttcggaaagtaaccctcgaaacaaattcatttgaaagaatgaaggaatgcaacnnnnnnnnnnnnnnnnnnnn

SEQ ID NO: 185 - RNA, 146 nt, synthetic construct
  source 1..146: mol_type = other RNA; note = Mature form sgRNA with modification of MS4-3/MS5-3 for TnpB
  misc_feature 127..146: note = n is a, c, g or u
cttcactgataaagtggagaaccgcttcaccaattagttgagtgaaggtgggctgcttgcatcagcctaatgtcgagaagtgctttcttcggaaagtaaccctcgaaacaaagaaaggaatgcaacnnnnnnnnnnnnnnnnnnnn

SEQ ID NO: 186 - RNA, 126 nt, synthetic construct
  source 1..126: mol_type = other RNA; note = Mature form sgRNA with modification of MS3-3/MS4-3/MS5-3 for TnpB
  misc_feature 107..126: note = n is a, c, g or u
accgcttcaccaattagttgagtgaaggtgggctgcttgcatcagcctaatgtcgagaagtgctttcttcggaaagtaaccctcgaaacaaagaaaggaatgcaacnnnnnnnnnnnnnnnnnnnn

SEQ ID NO: 187 - RNA, 10 nt, synthetic construct
  source 1..10: mol_type = other RNA; note = The additional sequence for TnpB gRNA
ataaaggtga

SEQ ID NO: 188 - RNA, 37 nt, synthetic construct
  source 1..37: mol_type = other RNA; note = The additional sequence for TnpB gRNA
ctgatgagtccgtgaggacgaaacgagtaagctcgtc

SEQ ID NO: 189 - RNA, 37 nt, synthetic construct
  source 1..37: mol_type = other RNA; note = The additional sequence for TnpB gRNA
ctgctcgaatgagcaaagcaggagtgcctgagtagtc

SEQ ID NO: 190 - DNA, 21 bp, synthetic construct
  source 1..21: mol_type = other DNA; note = Target Sequence for NLRC4
agagggagacacaagttgata

SEQ ID NO: 191 - DNA, 20 bp, synthetic construct
  source 1..20: mol_type = other DNA; note = Target Sequence for FUS
gtgggtaggtccagtttggg

SEQ ID NO: 192 - DNA, 20 bp, synthetic construct
  source 1..20: mol_type = other DNA; note = Target Sequence for LOC105370393
gcagtacacctgagggaaca

SEQ ID NO: 193 - DNA, 27 bp, synthetic construct
  source 1..27: mol_type = other DNA; note = Edit sequence
aacgtgacacgacgcgtttcggagaac

SEQ ID NO: 194 - DNA, 47 bp, synthetic construct
  source 1..47: mol_type = other DNA; note = shRNA for DCLRE1C
gcagagctctcgtttcacattcaagagatgtgaaacgagagctctgc

SEQ ID NO: 195 - DNA, 47 bp, synthetic construct
  source 1..47: mol_type = other DNA; note = shRNA for LIG4
gcatgatccttctgtaggattcaagagatcctacagaaggatcatgc

SEQ ID NO: 196 - DNA, 47 bp, synthetic construct
  source 1..47: mol_type = other DNA; note = shRNA for XRCC4
gaatccaccttgtttctgattcaagagatcagaaacaaggtggattc

SEQ ID NO: 197 - DNA, 47 bp, synthetic construct
  source 1..47: mol_type = other DNA; note = shRNA for KU70
gcagcattgtgcagatacattcaagagatgtatctgcacaatgctgc

SEQ ID NO: 198 - DNA, 47 bp, synthetic construct
  source 1..47: mol_type = other DNA; note = shRNA for XLF
gcatgagtctggcattacattcaagagatgtaatgccagactcatgc

SEQ ID NO: 199 - DNA, 47 bp, synthetic construct
  source 1..47: mol_type = other DNA; note = shRNA for ATM
gcaagcagctgaaacaaatttcaagagaatttgtttcagctgcttgc

SEQ ID NO: 200 - DNA, 51 bp, synthetic construct
  source 1..51: mol_type = other DNA; note = shRNA for Rad51
cgccaaagaaggagctaataattcaagagattattagctccttctttggcg

SEQ ID NO: 201 - DNA, 53 bp, synthetic construct
  source 1..53: mol_type = other DNA; note = shRNA for Scrambled
cagagctaactcagatagtactttcaagagaagtactatctgagttagctctg

SEQ ID NO: 202 - protein, 464 aa, synthetic construct
  REGION 1..464: note = TnpB homolog
MSIKAIRLEILKPYNEPDTATPVTWNELGQVLRDVRYACSKTENYAITKCYLWEQFKIEYKNNNGIFPNAKDFKEMTDLYSQLTAMFPDVAAAIVNQADQVATRKWNNEKKDVLSLRRSLTSFKLDVPIPIHNKSYKLRKISEDNKIIYVINVNLLSKKSERQTTYSMVLKVKDNSSKTILDRLINKELSPKGIQIIGSNKNRQKWFCLIPYDFTEKDTELNPDRIMGIDLGIAKAVYYAFSDSYKRGYIEGGEIEHFRKSVRARRIAIQNQGKYCGDGRIGHGVKRRLQPVEALREKEKNFRNLTNHRYARRLVEVAVKNHCGVIQMEDLTSITKDNTFLKDWPYYDLQTKIAEKASEYGIVFKKINPYKTSQRCSRCGYIDSENRPEQSVFVCRECGYGNMYLCEDCNKEQNHAGKCDSCGGVTNLITVNADYNAAKNIATKDIEQIIKKTMGKDYNPPKKK

SEQ ID NO: 203 - protein, 470 aa, synthetic construct
  REGION 1..470: note = TnpB homolog
MRIIRPYYGDEIEKFITAGKEKSKADGADGALTKIFWDRLKASHPEIVSAGEFYGLLCAMRMEAVVYYNRAISKLYQSLIVDVDGAQVSTAKALSAGPYHEFRERFTSYISLGLRQKLQSNFRRKELLRCQLALPTAKSDRFPIPISKQVDKQGKGGFKVSELQNGDFIIELPLMAYHKAKGKTEREYVELDAGPAILNIPVILSTQRRRANKTWFKDEGTDAEIRRVMSGEYKVSWLEILQRNRFGKAHGDWYVNFTIKYQPKDCGLDPKVKGGIDIGLSSPLVCAVTNSLDRLTIRDNDLVAFNKRALARRRTLLRRNRYKRAGHGSANKLEPITALTAKNELYRKAIMRRWAREAADFFRHNKAAAVNMEDLTGIKDREDYFSQMLRSYWNYSQMQTVLENKLKEYGIAVNYINPKDTSKTCHSCGHVNQHFDFSYRSANKFPMFKCVKCGVECGADYNAARNIAVA

SEQ ID NO: 204 - protein, 391 aa, synthetic construct
  REGION 1..391: note = TnpB homolog
MRDKLKASFAGEKLKKIKNAQISSPSATSDRFPIPMWQQTGFRVETNNEDLVIDIPFPLYKYREEVDKFKPWEKLEFIDTSKKKHIQLILSTNSRKRNVGWVKDWSTEAEIKRVMSKKLVINKIEITRGKRINERNYWFVNFVIAYEKPVRKLDSKITGGIDVGVSNPVVCAINSGLNRLTIRDNDVVDFTRAELARLRSQRRGDRFRRGGHGIKHKFKPSETIQKKYEQRRKKKMEEWASRITRFFLNNGVGLVYMENIDKKSISDGEDYFKVQLRVTWPVKEMQKLFERKLKENGIEVKSIDPKYSSQLCSKCGKWNTHFNFRYRQLNGYPPFECKYCDYGKDKEKEIIYADYNAARNLANPNFDKRRKVAIPSEVLKGNIKEEVVAEN

SEQ ID NO: 205 - protein, 424 aa, synthetic construct
  REGION 1..424: note = TnpB homolog
MKYTKVMRYQIIKPLNAEWDELGMVLRDIQKETRAALNKTIQLCWEYQGFSADYKQIHGQYPKPKDVLGYTSMHGYAYDRLKNEFSKIASSNLSQTIKRAVDKWNSDLKEILRGDRSIPNFRKDCPIDIVKQSTKIQKCNDGYVLSLGLINREYKNELGRKNGVFDVLIKANDKTQQTILERIINGDYTYTASQIINHKNKWFINLTYQFETKETALDPNNVMGVDLGIVYPVYIAFNNSLHRYHIKGGEIERFRRQVEKRKRELLNQGKYCGDGRKGHGYATRTKSIESISDKIARFRDTCNHKYSRFIVDMALKHNCGIIQMEDLTGISKESTFLKNWTYYDLQQKIEYKAREAGIQVIKIEPQYTSQRCSKCGYIDKENRQEQATFKCIECGFKTNADYNAARNIAIPNIDKIIRKTLKMQ

SEQ ID NO: 206 - protein, 424 aa, synthetic construct
  REGION 1..424: note = TnpB homolog
MKYTKVMRYQIIKPLNAEWDELGMVLRDIQKETRAALNKTIQLCWEYQGFSADYKQIHGQYPKPKDVLRYTSMHGYAYKHLKNEFSKIASANLAQTIKRAVDKWNSDLKEILRGDRSIPNFRKDCPIDIVKQSTKIQKCNDGYVLSLGLINREYKNELGRKNGVFDVLIKANDKTQQTILERIINGDYTYTASQIINHKNKWFINLTYQFEAKEAALDPNNVMGVDLGIVYPVYIAFNNSLHRYHIKGGEIERFRRQVEKRKRELLNQGKYCGDGRKGHGYATRTKSIELISDKIARFRDTCNHKYSRFIVDMALKHKCGIIQMEDLTGISKESTFLKNWTYYDLQQKIEYKAREAGIQVIKIEPQYTSQRCSKCGYIDKENRQEQATFKCIECGFKTNADYNAARNIAIPNIDKIIRKTLKMQ

SEQ ID NO: 207 - protein, 424 aa, synthetic construct
  REGION 1..424: note = TnpB homolog
MKYTKVMRYQIIKPLNAEWDELGMVLRDIQKETRAALNKTIQLCWEYQGFSADYKQIHGQYPKLKDVLGYTSMHGYAYDRLKNEFSKIASSNLSQTIKRAVDKWNSDLKEILRGDRSIPNFRKDCPIDIVKQSTKIQKCNDGYVLSLGLINREYKNELGRKNGVFDVLIKANDKTQQTILERIINGDYTYTASQIINHKNKWFINLTYQFETKETALDPNNVMGVDLGIVYPVYIAFNNSLHRYHIKGGEIERFRRQVEKRKRELLNQGKYCGDGRKGHGYATRTKSIESISDKIARFRDTCNHKYSRFIVDMALKHKCGIIQMEDLTGISKESTFLKNWTYYDLQQKIEYKAREAGIQVIKIEPQYTSQRCSKCGYIDKENRQEQATFKCIECGFETNADYNAARNIAIPNIDKIIRKTLKMQ

SEQ ID NO: 208 - protein, 427 aa, synthetic construct
  REGION 1..427: note = TnpB homolog
MLTKVMRYQIIKPLDDDWDVLGQVLRTVQRETHALLNKTIQLAWEWQGFSSEYKEKYGLYPIQQEILPKKKGGNVGSIMHYAYDQLKDIYTVSDRRNLNQSIKRATDKWKSDVPDIRKGEKSIPSFKKDCPIDVVSQAYSLHRGSEGFVMRAGLMSTEYKKELGRRFGSFDLLLNVKDNTQRTIIERLISGEYKAGVAQILRHKKDWFVNLTYSFEHVDSLLNPDRIMGVDLGIVYPVYLAFNDLFERYKIDGGEIESFRKQVERRRKQQNWQGKYCGDGRIGHGTHTRIKPTEVTEERIANFRDSCNHKYSRFVVEIALKHRCGTIQMEDLSGYSKATDDAFLKNWAYHDLQQKIEYKAKEVGIKVVKVKPECTSQRCSKCGHIAKENRQDREFLCKGCGFQVHADYNAARNIATKDIEEIIKQAL

SEQ ID NO: 209 - protein, 422 aa, synthetic construct
  REGION 1..422: note = TnpB homolog
MKHTKVMRYQIIKPINDTWETLGHVLREIQRETRAALNKTIQLAWEWQGFSAEYKQRYEEYPKTKDHLGYSALHGYAYNRLKDEFYRMNTANLSQTVKRAADKWKSDLKDVLRGDKSIASFKKDCPIDIVSQALRIRKDGSDYIMTLSLVSIKYRKELERKQSFFDVLISANDKTQRDILDRLIAGEYKLGASQLLYHKKKWFVNVNYQFEKEETAFDQDNIMGVDLGIVYPVYMAFNNSLNRYKIEGGEIERFRAQVERRKKQLLQQAKYCGDGRRGHGTKTRIQPIEVVSDKVANFRDTVNHRYSRYVVDMAIKHRCGTIQMEDLSGIAAEDTFLKRWSYYDLQQKIEYKAKEAGIQVVYIKPDYTSQRCSKCGHIERDNRTEQATFECKSCGFKTNADFNAARNIATKDIEKIIAETLK

SEQ ID NO: 210 - protein, 447 aa, synthetic construct
  REGION 1..447: note = TnpB homolog
MVKTMKFQIIKPINMLWKDFENILRQLQQDTRNIKNKTIQLCWEYQGFSSEYKEKHGEYPKHSDILNYKTITGYIYDRLNNEYYRLNTGNLSDTIKSATDKWRNDIVDILKGEVSIPSYKRDAIIHVKNTNYKIVPEDGRYYLRLSLLSNVYRKELDLEKGQIDVAIRVADKNQKVTLERIFSGEYKQSSSQLMKKKNKWFFYMAFKFDPKTAKDLDPNNVMGIDMGITHPIYFAFNNSLKRGKIEGGEVESFRRRVEQRRRELLAQGKYCGKGRRGRGYETRVKPIKRIGDKIERFKDTANHKYSRYIVDVAVKNNCGIIQMEDLKGISKNNIFLKNWPYFDLQTKIEYKAKEKGIVVKKIAPRYTSQRCSKCGYINKENRVSQDTFKCVKCDFGHKFYVNADYNAARNIATPGIEEIIKKQIEKQKEMDEWENETIKLPLVGSDK

SEQ ID NO: 211 - protein, 411 aa, synthetic construct
  REGION 1..411: note = TnpB homolog
MTKAKDRELSKVFRVEVLKPLNLTWDEFGGLLRRTQYHAAHLANEVITTQYLLAKGKLERNGSFCALVAHACHDCSLHADVKCTVCKWARDKFKADARRILRADISLPSYKNNLCMIKNRSVKLRETPDGWAARLAILPKADGKNQVQPEVLLRTEEMKRRSPGAYQVLERIASKEYKQGTTQVKRDTRTGKIYLLISYSFRPERESGLEASRVMGVDLGVSTPAYCAFNDSLKRKSLLIEGRKLLKTKWQIEGRRRDIRRHNDQRDLRRGHGKEAKFRPMEAVEQHWVDFRQSWNHVLARRIIEYALSNHAGAIHLEDLSPGTNSKFLGRNWPVAELLDYIEYKAKERGIAVKRVNPFKTSQTCSDCGAIKESFTFGDRKKAGFPDFVCDACGFRTHADYNAARNIAKAP

SEQ ID NO: 212 - protein, 429 aa, synthetic construct
  REGION 1..429: note = TnpB homolog
MVKVVKIYLISEQVDEQGKDVDYNTICGVLWDLQWETREIKNKTVQLCWEWSGFSSDYYKKYGEYPKEKNLLDYTMGGFVYDKLKSKYHLYTANLSTTSQNTCGIFRTYKVDFVKGNRSVLSFKADQPLDVHKKSISIDRIDDNYFVKLKLLNKSGIQKYGIRDDFHFRMLVKDNSTKTILERCVGGDYKAAASKIIYDKKKKMWCLNLSYEFDVNTAKDLNKNRILGIDIGIVYPVVASVNGELDRFVIQGGEIETFRRRVENRKKSLLKQTKYCGDGRIGHGRNKRTEPVDIISDQIARFRNTANHKYSRAVIDYAVRKQCGTIQMENLKGITDKSDRFLKNWSYYDLQQKIEYKAKEKGINVVFINPKYTSQRCSRCGYIDSANRPKLPNQSKFLCIKCGFTENADYNASQNIALYNIEKLIDAEA

SEQ ID NO: 213 - protein, 433 aa, synthetic construct
  REGION 1..433: note = TnpB homolog
MGKGVLAKVMKYELRYLDGCGDFSNMQEQVWALQRQTREILNRSIQIAFQWDCANSEHHRKTGEYLDLKTETGYKRLDGHIYNCLKGQYEDMATSNLNATIQKAWKKYNSSKKEILRGSMSIPSYKMNQPLTLDKNTVKLSEGERNPIVTLTLFSDKFKRAQGVSNVKFSMPLHDGTQRAIFANLMNGTYQLGECQLVYKRPKWFLFVTYKFPPVEHPLDPDKILGVDMGEACALYASTFGEHGYLKIDGGEITKYAKKMEARIRSMQKQAAHCGEGRIGHGTKTRVSVVYQAKDKVARFRDTINHRYSKALIDYALKNQCGTIQMEDLTGIKEDTGFPKFLRHWTYYDLQSKIEAKAAEHGIQVVKINPRHTSQRCSRCGHIDKANRTSQADFCCTKCGFSANADFNASQNISIRNIDKIIAKAIGANRKQT

SEQ ID NO: 214 - protein, 438 aa, synthetic construct
  REGION 1..438: note = TnpB homolog
MGKVHTRTIKLKLIVSTEDKNVAWKRIRQISNDAWRAANWIASGQLFNDQLVRRIYARRKINPREDSEAVEQIEKEFEAFFGTKRQATTEWDIKEAFPDLPPYVTNPLNHVVVASYKKEKPDMLSGNRSLRTYKRGMPIQTAKAAINFSKNETGQHFVKWTLGRKEFIDFEIYYGQDRANNRLTIDRIINGQIDYSAPMIQLKDKNLFLLLPVKEPEIAADLDPDIALGVDLGVATPAYMALSKGPARRAVGDKEDFLKVRLQMQSRKRRLQRSIKSAHGGKGRQKKLKALNQIGEKERQFARTYNHYISREIVNFAIRHNAGTIKLEMLEGFGQEEQQAFVLRNWSYFELQTFIEYKAKKVGIKILKIDPYRTSQTCSSCGHFEEGQRKDQSTFECKNCGEKLHADYNAALNIARSKKIVTKKEQCEYYLNRNQNTI

SEQ ID NO: 215 - protein, 433 aa, synthetic construct
  REGION 1..433: note = TnpB homolog
MVCNKVVKIALICDQIDKDGKDVNYNDIYKLLWDLQKQTREAKNKVIRLCWEWSGYSSEYFKTHEEYPKDKEIFGISLRGYLYDRIKGDYNLYSGNLSQSAEIAYKEYKNSLKDVLRGDKSIINYRENQPLDIKNKAIQLLYENDNFFVRVALINKDKQKELNFKDCSVRFKLLVKDDSTRTILERCFDEVYTITASKIMYNKKKKQWYINLGYKFTKEIDKTLDKDRILGVDLGVINPLVASVYGSYDRLIIGGGEIDKFRKRVEANKVQMLKQGKYCGDGRIGHGVNTRNKPAYNIEDKISRFRDTVNHKYSKAVVDYAVKNNCGTIQMEDLKGITQNKNERYLKNWTYFDLQTKIEYKAKALGIEVKYKNPKYTSQRCSKCGHIAEENRPEQKTFKCVKCGFKVNADYNASQNLAIKDIDKIIEQYYNKG

SEQ ID NO: 216 - protein, 433 aa, synthetic construct
  REGION 1..433: note = TnpB homolog
MVCNKVIKIALICDQIDKDGKDVNYNDIYKLLWDLQKQTREAKNKVIRLCWEWSGYSSEYFKTHEEYPKDKEIFGISLRGYLYDRIKGDYNLYSGNLSQSAEIAYKEYKNSLKDVLRGDKSIINYRENQPLDIKNKAIQLLYENDNFFVRVALINKDKQKELNFKDCSVRFKLLVKDDSTRTILERCFDEVYTITASKIMYNKKKKQWYINLGYKFTKEIDKTLDKDRILGVDLGVINPLVASVYGSYDRLIIGGGEIDKFRKRVEANKVQMLKQGKYCGDGRIGHGVNTRNKPAYNIEDKISRFRDTVNHKYSKAVVDYAVKNNCGTIQMEDLKGITQNKNERYLKNWTYFDLQTKIEYKAKALGIEVKYKNPKYTSQRCSKCGHIAEENRPEQKTFKCVKCGFKVNADYNASQNLAIKDIDKIIEQYYNKG

SEQ ID NO: 217 - protein, 433 aa, synthetic construct
  REGION 1..433: note = TnpB homolog
MVCNKVVKIALICDQIDKDGKDVNYNDIYKLLWDLQKQTREAKNKVIRLCWEWSGYSSEYFKTHEEYPKDKEILGISLRSYLYNRIKGDYNLYSGNLSQSAKIAYIEYKNSLTDVLRGDKSIINYRENQPLDIKNKAIQLLYENDNFFVRVALINKDKRKELNFKDCSVRFKLLVKDDSTRTILERCFDEVYTITASKIMYNKKKKQWYINLGYKFTKEIDKTLDKDRILGVDLGVINPLVASVYGSYDRLIIGGGEIDKFRKRVEANKVQMLKQGKYCGDGRIGHGVNTRNKPAYNIEDKISRFRDTVNHKYSKAVVDYAVKNNCGTIQMEDLKGITQNKNERYLKNWTYFDLQTKIEYKAKALGIEVKYKNPKYTSQRCSKCGHIAEENRPEQKTFKCVKCGFKVNADYNASQNLAIKDIDKIIEQYYNKG

SEQ ID NO: 218 - protein, 438 aa, synthetic construct
  REGION 1..438: note = TnpB homolog
MQKVLKVYLICEQLDPDGSPVDYKDIFKLLWDLQKQTREIKNKSIQYCWEFSNFSSDYYKEHHEYPKDKEILNYTLGGFVNDKFKTGNDLYSANCSTTVRTACAEFKNAKADFMRGEKSIISYKANQPLDLHNKSIRLEYQKGTFLFYLKLLNRSAVKKHGFQSSEIRFKAIVKDNSSQTILERCTAGVYDMAASKLLYDQKKKCWVLNLVYAFEPETPEALDPEKILGVDLGVHYPICASVYGDLKRFIIDGGEIESFRKRVEARKISMLKQGKNCGGGRIGHGIQTRNKPVYAIADKIARFRDTVNHKYSRALIDYAIKNNCGVIQMEKLTGVTADANRFMKNWTYFDLQTKIEYKAQEAGIQIVYIEPKYTSQRCSKCGYIDRENRPEQSKFICRKCGFSENADYNASQNIGIRNIEKLIEKQLQTKCESETDTT

SEQ ID NO: 219 - protein, 440 aa, synthetic construct
  REGION 1..440: note = TnpB homolog
MVKVVKIYLISEQFDKAGNRIDYKEVNKILWELQKQTREAKNKTVQLLWEWNNFSSDYVKASGIYPKAKDIFGYSSVHGQANKELRTKLILNSSNLSTTTMDVCKIFNTYKKEVWEGKRSVPSYKSDQPLDLHKDSIKLIYENNQFYVRLALLKKAEFAKYGFKDGFRFKMQVKDNSTKTILERCFDEVYKINASKLLYDQKKKMWKLNLSYSFDNKNISELDKEKILGVDVGVNCPLVASVFGDRDRFIIKGGEIEKFRKSVEARRRSMLEQTKYCGDGRIGHGRKKRTEPALNIGDKIARFRDTTNHKYSRALIEYAVKKGCGTIQMEKLTGITSKSDRFLKDWTYYDLQTKIENKAKEVGINVVYIAPKYTSQRCSKCGYIHKDNRPNQAKFRCLKCDFESNADYNASQNIGIKNIAKIIEKDLKKQKSEVQVNENK

SEQ ID NO: 220 - protein, 332 aa, synthetic construct
  REGION 1..332: note = TnpB homolog
MAIPVRCDKPGQKRLEKTNDGQVEVDLMICTHPYPRVVLATQDKSLGKGARTILAHLLENKDQSKNGYRQRYFEIKEDKLSHKWFLLVSYDFPASTPSLSKERIVGVDLGISCPLYVAINNGYARLGWRQFHALAARIRAIQNQTIRRRREILRGGKTIISDDRARSGHGLKRKLLPIEKLQGRIDRAYTTINHQFSSAVIKFAKDHGAGMIQIEDLDGLKEILSGTFLGERWRYSELQQFIKYKAKENGIEVKEVNPQYTSQRCSQCGYINEQFTFNYRQEQRQKLGKPVPFTCPECKYEANADYNAARNLATLDIEQLIMRQLDKQGIKN

SEQ ID NO: 221 - protein, 424 aa, synthetic construct
  REGION 1..424: note = TnpB homolog
MATKVMRYQIIKPIDCNWDLFGKVLRDIQYDTRQIMNRTIQYCWEWQGYSSDYKIAKGEYPKTRETFGYSDMRGYAYDKLKSIYQRLNTANLTTSITRAVQRWKTDTKDVIRGDKSIACFRADVPIDLHNKSMNIEKSDDGYIVALSLASNIYKKELDRNSGQFSVLINEGNKSNRDVLDRCIAGQYKISASQILREKNKWFLNLSYSFEISKPDKSRDNILGIDVGIVHPVYMAVYNSPARRSISGGEIDNFRKQVQKRIKELQLQGKQCGEGRIGHGIKTRVKPIEFAKDKVANFRNTINHKYSKAIVEFAIKNGCGIIQMEDLKGINTDNVFLKNWTYYDLQQKVKYKAELEGIEVKLIDPQYTSQRCCKCGYIHRDNRPEQAKFKCIDCGFEVNADYNASLNIATPDIDKIILEFLKCET

SEQ ID NO: 222 - protein, 440 aa, synthetic construct
  REGION 1..440: note = TnpB homolog
MVKVVKIHLISEQFDKAGNRIDYEEVNKILWELQKQTREAKNKTVQLLWEWNNFSSDYVKASGIYPKAKDIFGYSSVHGQANKELRTKLALNSSNLSTTTMDVCKNFNTYKKEVWKGKRSVPSYKSDQPLDLHKDSIKLIYENNEFYVRLALLKKAEFAKYGFKDGFRFKMQVKDNSTKTILERCFDEVYKINASKLLYDQKKKKWKLNLSYSFDNKNISELDKEKILGVDVGVNCPLVASVFGDRDRFIIKGGEIEKFRKSVEARRRSMLEQTKYCGDGRIGHGRKKRTEPALNIGDKIARFRDTTNHKYSRALIEYAVKKGCGTIQMEKLTGITSKSDRFLKDWTYYDLQTKIENKAKEVGINVVYIAPKYTSQRCSKCGYIHKDNRPNQAKFRCLECDFESNADYNASQNIGIKNIDKIIEKDLQKQESEVQVNENK

SEQ ID NO: 223 - protein, 436 aa, synthetic construct
  REGION 1..436: note = TnpB homolog
MNKVVRLALICEHSDKDGNPVDYSDVYKLLWQLQAQTREIKNKTIQYCWEYSNFSSDYYKENHEYPKEKDVLHYALDGFVNDKFKVGNDLYSSNCSYMTRKVCAEFKKSKSDFLKGTRSIISYKSNQPLDLHNKSIRIEYKDNDFFAFLKLLKRPAFNRLGYKNSEIGFKVIVRDKSTRTILERCVDQIYGISASKLIYNKKKKQWFLNLVYAFEPDNANNLDPSKILGVDLGIHYPICASVYGDLQRFTIHGGEIEEFRRRVESRKLSLLKQGKNCGDGRIGHGGKTRNKPVYSIEDRIARFRDTVNHKYSRALIDYAVKKECGTIQMEDLSGITAESDRFLKNWSYYDLQSKIEYKAKEKGIKIVYIDPKYSSQRCSKCGHIDKENRKTQSSFVCLKCGFEENADYNASQNIGIKDIDKIIENDLSSKCETDVN

SEQ ID NO: 224 - protein, 439 aa, synthetic construct
  REGION 1..439: note = TnpB homolog
MKPMNKVVRLALICEHSDKDGNPVDYSDVYKLLWQLQAQTREIKNKTIQYCWEYSNFSSDYYKENHEYPKEKDVLHYALDGFVNDKFKVGNDLYSSNCSYMTRKVCAEFKKSKSDFLKGTRSIISYKSNQPLDLHNKSIRIEYKDNDFFAFLKLLKRPAFNRLGYKNSEIGFKVIVRDKSTRTILERCVDQIYGISASKLIYNKKKKQWFLNLVYAFEPDNANNLDPSKILGVDLGIHYPICASVYGDLQRFTIHGGEIEEFRRRVESRKLSLLKQGKNCGDGRIGHGGKTRNKPVYSIEDRIARFRDTVNHKYSRALIDYAVKKECGTIQMEDLSGITAESDRFLKNWSYYDLQSKIEYKAKEKGIKIVYIDPKYSSQRCSKCGHIDKENRKTQSSFVCLKCGFEENADYNASQNIGIKDIDKIIENDLSSKCETDVN

SEQ ID NO: 225 - protein, 440 aa, synthetic construct
  REGION 1..440: note = TnpB homolog
MVKVVKIHLISEQFDKAGNRIDYEEVNKILWELQKQTREAKNKTVQLLWEWNNFSSDYVKASGIYPKAKDIFGYSSVHGQANKELRTKLALNSSNLSTTTMDVCKNFNTYKKEVWKGKRSVPSYKSDQPLDLHKDSIKLIYENNQFYVRLALLKKAEFAKYGFKDGFHFKMQVKDNSTKTILERCFDEVYKINASKLLYDQKKKKWKLNLSYSFDNKNISELDKEKILGVDVGVSYPLVASVFGDRDRFKIKGGEIEKFRKSVEARRRSMLEQTKYCGDGRIGHGRKKRTEPALNIGDKIARFRDTTNHKYSRALIEYAVKKGCGTIQMEKLTGITSKADRFLKDWTYYDLQTKIENKAKEVGINVVYIAPKYTSQRCSKCGYIHKDNRPNQAKFRCLECDFESNADYNASQNIGIKNIDKIIEKDLQKQESEVQVNENK

SEQ ID NO: 226 - protein, 439 aa, synthetic construct
  REGION 1..439: note = TnpB homolog
MVKVVKIHLISEQFDKAGNRIDYKEVNKILWELQKQTREAKNKTVQLLWEWNNFSSDYVKASGIYPKAKDIFGYSSVHGQANKELRTKLALNSSNLSTTTMDVCKNFNTYKKEVWKGKRSVPSYKSDQPLDLHKDSIKLIYENNQFYVRLALLKKAGFAKYGFKDGFRFKMQVKDNSTKTILERCFDGIYTIVASKLLYDQKKNRWKLNLSYSFDNKNISELDKEKILGVDVGVSYPLVASVFGDRDRFKIKGGEIEKFRKSVEARRRSMLEQTKYCGDGRIGHGRKKRTEPALNIGDKIARFRDTTNHKYSRALIEYAVKKGCGTIQMEKLTGITSKSDRFLKDWTYYDLQTKIESKANEAGIKVVYIAPEYTSQRCSKCGYIHKDNRPNQAKFRCLKCDFESNADYNASQNIGIKNIDKTIKKERKKQKSEAQVNEK

SEQ ID NO: 227 - protein, 429 aa, synthetic construct
  REGION 1..429: note = TnpB homolog
MTKVIKLALICQQSDSNGMPVDYKEVNKILWELQRQTREIKNKSIQYCWEYHNFSSDYYKRNGEYPKEKDVLLFTLGGYVNDKFKTGNDLYSANCSTTVRGVCGEFKNSKKDFISGKRSIISYKENQPLDLHNKSIRLEYSDHEFYVYLKLLNRQGFKKFNFADTQIMFKILVRDNSTKTILERCLDEVYSVSASKLIYDKKKKCWVLNLSYSFSGEITHNLDENRILGVDLGIHYPICASVYGEWKRFTIDGGEIEEYRRRVEARKKTLLKQGKNCGDGRIGHGVKTRNKPVYSIEDRISRFRDTANHKYSRALINYAIKNNCGVIQMENLEGVTAHSDKFLKNWSYYDLQTKIEYKAKEAGIKVVYINPRYTSQRCSKCGYTDTDNRPEQAKFICKKCGFSENADFNASQNIGIKNIEQIIKEEIQI

SEQ ID NO: 228 - protein, 422 aa, synthetic construct
  REGION 1..422: note = TnpB homolog
MMTKSVKIKLGTPIDSNWNTVRKILADLRYNSSKMLNFSIQQCYQWMIYRNEYREKYGKYPRAKDIYGYSHRNHIYRQAAEIFPIFNRGNISQTVGMATSRWSSDQKDVMSLRKSIPSYRLQAPIYIANQSYTISRTENGLVVDCSLVSKKYAKEETNDKTRYRISLVVKDNSTETILDRIVSGEYSQGYGQIVKDRRKEKWYLLVAYRFEPKKTKETGRILGIDLGIVYPLYMALNDSHHRYRIDGGEIEHFRRNIEKRKNQLLDQGKYCGDGRRGHGIRTRIAPIEFAREKIKNFRNTTNHKYSKFVVDIAQKHDVETIQLEKLDGISEDSTFLKNWSYYDLQQKIQYKAQEKGIKVAYIDPRYTSQRCSRCGNISRENRQDQQRFRCTKCGFSANADYNAAKNISTQNIEKIIEEELKK

SEQ ID NO: 229 - protein, 443 aa, synthetic construct
  REGION 1..443: note = TnpB homolog
MTLLVKVVKIYLISEQFDKAGNRIDYKEVNKILWELQKQTRKAKNKTVQLLWEWNNFSSDYVKASGIYPKAKDIFGYSSVHGQANKELRTKLALNSSNLSTTTMDVCKIFNTYKKEVWEGKRSVPSYKSDQPLDLHKDSIKLIYENNEFYVRLALLKKAEFAKYGFKDGFRFKMQVKDNSTKTILERCFDEVYKINASKLLYDQKKKMWKLNLSYSFDNKNISELDKEKILGVDVGVSCPLVASVFGDRDRFIIKGGEIEKFRKSVEARRRSMLEQTKYCGDGRIGHGRKKRTEPALNIGNKIARFRDTTNHKYSRALIEYAVKKGCGTIQMEKLTGITSKSDRFLKDWTYYDLQTKIENKAKEVGINVVYIAPKYTSQRCSKCGYIHKDNRPNQAKFRCLECDFERNADYNASQNIGIKNIDKIIEKDLKKQKSEVQVNENK

SEQ ID NO: 230 - protein, 436 aa, synthetic construct
  REGION 1..436: note = TnpB homolog
MNKVVRLALICEHFDKDGNPVDYSDVYKLLWQLQAQTREIKNKTIQYCWEYSNFSSDYYKENHEYPKEKDVLNYTLGGFVNDKFKVGNDLYSANCSTTTQTVCAEFKNSKSEFLKGTKSIINYKSNQPLDLHNKSIRVEYKDNDFFVFLKLLNRHAFKRLGYKNTEICFKVIVRDKSTRTILERCVDQIYGISASKLIYNKKKKQWFLNLVYAFEPDNANNLDPNRILGVDLGIHYPICASVYGDLQRFTIHGGEIEEFRRRVESRKLSLLKQGKNCGDGRIGHGVKTRNKPVYSIEDRIARFRDTVNHKYSRALIDYAVKKECGTIQMEDLSGITAESDRFLKNWSYYDLQTKIEYKAKEKGIKIVYIDPKYSSQRCSKCGHIDKENRKTQSSFVCLKCGFEENADYNASQNIGIKDIDKIIESDLSSKCETDVN

SEQ ID NO: 231 - protein, 440 aa, synthetic construct
  REGION 1..440: note = TnpB homolog
MVKVVKIHLISEQFDKAGNRIDYKEVNKILWELQKQTREAKNKTVQLLWEWNNFSSDYVKASGIYPKAKDIFGYSSVHGQANKELRTKLILNSSNLSTTTMDVCKIFNTYKKEVWEGKRSVPSYKSDQPLDLHKDSIKLIYENNQFYVRLALLKKAEFAKYGFKDGFRFKMQVKDNSTKTILERCFDEVYKINASKLLYDQKKKMWKLNLSYSFDNKNISELDKEKILGVDVGVNCPLVASVFGDRDRFIIKGGEIEKFRKSVEARRRSMLEQTKYCGDGRIGHGRKKRTEPALNIGDKIARFRDTTNHKYSRALIEYAVKKGCGTIQMEKLTGITSKSDRFLKDWTYYDLQTKIENKAKEVGINVVYIAPKYTSQRCSNCGYIHKDNRPNQAKFRCLKCDFESNADYNASQNIGIKNIAKIIEKDLKKQKSEVQVNENK

SEQ ID NO: 232 - protein, 439 aa, synthetic construct
  REGION 1..439: note = TnpB homolog
MFMTKVTKVYLISEQIDKDGNKIDFKKISELLWNLQRQTRDIKNKCVQLCWEWLNFSSDYYKKSEEYPKEKDTLGYTLSGFVYDRIKNGSDLYSSNLSTSSRDTCTAFSNYKKEMLNGERSVLSFKANQPLDIHNKAIKLSYENGNFFVALKMLNRAGKEKYGINDDLRFRMQVRDKSVRTILERLMNDEYKVSASKLMYDKKKKLWKLNLCYSFDNHVISTLDPEKIMGVDLGVVYPIMASVNGDYARFSIKGGEIEAFRNRVEARRRSLLNQSRYCGDGRIGHGRKKRTEPAAQIADKIARFRDTTNHKYSRALIDYAIKNGCGTIQMEKLTGITSNAEHFLKEWSYFDLQTKIESKAKEAGIKVVYINPKFTSQRCNKCGYIHTDNRPVQARFCCQKCGYEENADYNASQNIGTKHIDVIIEETLKMQCEPEVPTE

SEQ ID NO: 233 - protein, 434 aa, synthetic construct
  REGION 1..434: note = TnpB homolog
MNENMCALTKIMKYELRYLDGFPDFSAMQNAVWPLQRQTREILNRTIQEAYHWDYFSATKKKETGEYPDLLKETGYKRLDGYIYHVLAPDYPDFSSSGVNATIQKAWKKYKSSRADVWKGEMSLPSYKSDQPIVLHAKQIKLSGDNRAAAVTLSLFSNKFKKEHAISGNVQFAITLHDNTQRTIYQKLRNGEYKLSESQLVYDKKKWFLYLAYSFNPAEHALDPEKILGVDMGEKFALYASSFGEYGHFKIEGSEVTEYAKALERRRRSLQQQARYCGEGRIGHGTKTRVGAVYREEDRIANFRSTINHRYSKALIEYAVKNGYGTIQMENLTGIKENLQFPRRLQHWTYYDLQSKIEAKAKEHGIAVVKVNPKHTSQRCSRCGHIAAENRPKQEVFQCVKCGYACNADFNASQNISIKDIEKLIQETIGANPK

SEQ ID NO: 234 - protein, 475 aa, synthetic construct
  REGION 1..475: note = TnpB homolog
MKEKYFVKVAKFEILKPANGMTWKEFRQLLMSVRYRVFRLANLCVSENFLQFHLWRKKEIDKIPTLKISELNRQLREMLLEEKKTSDAEQTRICKRGALPASIVDALSQYKIRALTAKSKWRDVIRGNASLPSFRNDAAIPICCHKPSHRRLEKTSNGNVELELMICMKPYPRIILKTEKISGNMKATLERLLANRGNSDTGYQQRFFEVVQDRQEGRRWYLHVTYKFPASLLRLNPQVIVGIDLGFSCPLYAAINNGLARLGWRHYESLGKRIRNLQNQVFARRRSMQSGGNASLTMDTARGGHGRKRILRPIEKLAGRVNNAYSTLNHQLSRSVIEFAKNHGAGVIQMENLEGLKEQLTGTFLGSRWRYHELQQFIEYKAKEVGIEVRKINPQYTSRRCSECGYINIKFDRAFRDANRKDGKTAKFICPKCKWEGDPDYNAARNLATLDIENLIRQQLINQGIPSEREETPVL

SEQ ID NO: 235 - protein, 430 aa, synthetic construct
  REGION 1..430: note = TnpB homolog
MCALTKIMKYELRYLDGFPDFSAMQNAVWPLQRQTREILNRTIQEAYRWDYFSATKKKETGEYPDLQKETGYKRLDGYIYHVLSPDYPDFSSSGVNATIQKAWKKYKSSKADVWKGEMSLPSYKSDQPIVLHAKQIKLSGDTRAAAATLSLFSNKFKKEHEISGNVQFAITLHDNTQRTIYQKLRNGEYKLSESQLVYDKKKWFLYLAYSFNPAEHALDPEKILGVDMGEKFALYASSFGEYGHFKIEGSEVTEYAKALERRRRSLQQQARYCGEGRIGHGTKTRVGVVYREEDRIANFRSTINHRYSKALIEYAVKNGYGTIQMENLTGIKENLQFPRRLQHWTYYDLQSKIEAKAKEHGIAVVKVNPKHTSQRCSRCGHIAAENRPKQEVFQCVKCGYACNADFNASQNISIKDIEKLIQETIGANPK

SEQ ID NO: 236 - protein, 450 aa, synthetic construct
  REGION 1..450: note = TnpB homolog
MSTVVKVMKYQIVCPVNIEWKVFETYLRTLTYQVRTIGNRTIQKLWEFDNQSLNHFKENGVYPSTQQLYGCTQKTISGYIYDQLKFEYLDINKANMSTTLQKTIKTWNSRKKEIWSGEMSIPSFRNNLPIDIHGNSIQLTKEKSGDYIANLSLFSSSFIRENELSSGKILVKLSTRKQNSMKVILDRLIDGTYAKGASMLHKYKNKWYLSVTYKANAIEESKFDEDFIMGIDMGKVNVLYFAFNKGFIRGSISGEEIEDFRKKIEHRRISLLRQGKYCSENRIGKGRKKRIKPVDVLNDKVARFRNSTNHKYANYIVQQCLKYKCGCIQLENLQGISKEQTFLKNWTYFDLQEKIENQANQYGIKVVKIAPSYTSQRCSECGYIHKNNRQDQSTFECQQCNLKVHADYNAAKNISIYNIEKLIQKQLKLQEKLNSKKYTEQYKEQIENIT

SEQ ID NO: 237 - protein, 439 aa, synthetic construct
  REGION 1..439: note = TnpB homolog
MFMTKVTKVYLISEQIDKDGNKIDFKKISELLWNLQMQTRDIKNKCVQLCWEWLNFSSDYYKKSEEYPKEKDTLGYTLSGFVYDRIKNGSDLYSSNLSTSSRDTCTAFSNYKKEMLKGERSVLSFKANQPLDIHNKAIKLSYENGNFFVALKMLNRAGKEKYGIKDDLRFRMQVRDKSVRTILERLMNDEYKVSASKLMYDKKKKLWKLNLCYSFDNHVISTLDTEKIMGVDLGVVYPIMASVNGDYARFSIKGGEIEAFRSRVEARRRSLLNQSRYCGDGRIGHGRKKRTEPATQIADKIARFRDTTNHKYSRALIDYAIKNGCGTIQMEKLTGITSNAEHFLKEWSYFDLQTKIESKAKEAGIKVVYINPKFTSQRCNKCGYIHTDNRPVQARFCCQKCGYEENADYNASQNIGTKHIDVIIEETLKMQCEPETPTE

SEQ ID NO: 238 - protein, 436 aa, synthetic construct
  REGION 1..436: note = TnpB homolog
MNKVVRLALICEHFDKDGNPVDYSDVYKLLWQLQAQTREIKNKTIQYCWEYSNFSSDYYKENHEYPKEKDVLNYTLGGFVNDKFKFGNDLYSANCSTTTQTVCAEFKNSKSEFLKGTKSIINYKSNQPLDLHNKSIRVEYKDNDFFVFLKLLNRPAFNRLGYKNSEICFKVIVRDKSTRTILERCVDQIYGISASKLIYNKKKKQWFLNLVYAFEPDNANNLDPNKILGVDLGIHYPICASVYGDLQRFTIHGGEIEEFRRRVESRKLSLLKQGKNCGDGRIGHGVKTRNKPVYSIEDKIARFRDTANHKYSRALIDYAIKKECGTIQMEDLSGITAESERFLKNWSYYDLQTKIEYKAKEKGIKIVYIDPKYSSKRCSKCGYIDRENRKTQSSFVCLKCGFEENADYNASQNIGIKDIDKIIENDLSSKCETDIT

SEQ ID NO: 239 - protein, 427 aa, synthetic construct
  REGION 1..427: note = TnpB homolog
MVLTRKLQLVPCAEGMSKEEAKKEVDRVYKILRDGIYAQNKAYNIFISRRYTAILLGASKEELAKLTLIGERNPKKDDPSYSLYEYGKINFIKGIPQASALGQHAISDLSKQKKDGLFKGKVALACRRLDAPMWIKQKYEFYHNYADNKELSENLYSEDLKIYMKLANICVFEVVLGNPHKSAAIRAELERVFDENYKKLDSSIQIVNNKIMLYLAINIPEKQIELKEDVVVGVDLGIAIPAVCALNNSRYIKKSIGSANEFLRIRTQLQSEKKRLQRKLRDTNGGHGRKKKLAPLDKLSKRERNFVQTYNHMISRRVVDFAVKNNAKYINVEDLSDYKNNGSEYILRNWSYYELQQQIEYKAEMYGIVVRKVNPYHTSQICSQCGHWEEGQRKSQSEFECKACGYTANADFNAARNIALSTDFVKK

SEQ ID NO: 240 - protein, 433 aa, synthetic construct
  REGION 1..433: note = TnpB homolog
MSKGVVTKVMKYTLRYIGGCGDFHKMQEAVWKLQRQTREVLNKTVQLAFDWDHRSREAYRTSGEYLDIVKETGYKRLDGYIYNRLKTDYADFASSNLNATIQVAWKKYMASKSDILTGKMSFPSYKSNQPIVLHNSSIRFSTEKYGVPAAELTVFSNALKKENGLSTNPAFEILLMDGTQRSIFQRVISGEYKHGQCQINYEKRKWFLYLTYTFEAGKTPLDPDKILGVDIGETLAICASSTSEWGRFVIQGGEVTRYSKQIEERRRSQQRQATYCGEGRIGHGTKARVAPIYATEDRIANFRDTINHRYSKALIEYAVKHGFGTIQMEDLSGIKGEKDFPKFLRHWTYYDLQNKIEAKAKEQGINVVKVQPAYTSQRCSKCGCIDKENRKNQELFCCVKCGFKANADFNASQNISIKGIDKIIEKEYNANIE

SEQ ID NO: 241 - protein, 424 aa, synthetic construct
  REGION 1..424: note = TnpB homolog
MPTRVMKYQIVKPMNCDWKLLNRHLLDLQQEAHQILNKTIQLCWEWQGFCSEYKAKYDIYPVDKDIFHLTLAGYVNRMLRLQFPKSNSNNLGTSRIKAINRWHTDLKDVKSGQKSIASFKADVPIDLHYLSIKLHKEKDCYYADLSLISNIYKKELGRESGKLLVLLKSGDEVSRDILRNCLDGIYKIRASDISHKKNKWFLNLHYNYEETNKSLDKDRILGIDMGIAYPVYMSVYNTQITSYIEGGEIERFHKQVEKRSAEFQRQGKYCGNGRIGHGVKTRLKPLSFATDKIANFRETTNHKYSKYIVDFAVKNNCGNIQMEDLTGIKNERIFLRNWTYFDLQKKIRYKAEENGINVLLIKPHYTSQRCSQCGDIDKKSRITQENFTCISCGYQTNADHNASINISTPNIENIINDFMSLKID

SEQ ID NO: 242 - protein, 437 aa, synthetic construct
  REGION 1..437: note = TnpB homolog
MNKVVKLALISKVKDKDGNDVKYGDVCKILWELQRQTREIKNKAVQFCWEWNGFSSEYNNLFGEYPKDKDYLKNKSEGKPIVLRSFVYDRLKSDYYLNSSNLSTTTSLAFKEFKQYLTDIRKGERSVLNYKNNQPLELHNECIWLESNNGKFITRFSFLNKAGKDFYSIDNFTFEVIVKDNSTKTILERCIDSIYGIRASKLIYNQKKKQWFLNLSYSFEAKEIATLDKDKILGVDLGIALPICASVYGDLDRFTIKGGEIEHFRKSIESRKRSLLQQGKVCGDGRIGHGIHTRNKPAYNIEDKIARFRDTANHKYSRALIDYAVRKGCGTIQMEMLKGITEEKDPFLKNWTYFDLQQKIEYKAKEKGIKVVYIAPKYTSRRCSKCGHIDKDNRLTQANFLCLNCGYKENADYNASQNIAIKDIDKIIIEETKGGES

SEQ ID NO: 243 - protein, 463 aa, synthetic construct
  REGION 1..463: note = TnpB homolog
MTCTKTMRYQIVRPLDDDWEVFRYILNQISYETWNCLNRCAQYLWEADNFKKIYYSKFGIKFNVKDVEGVADDAYINRNLKKEFQKMNGDSVETITREVKVKMKKNKEDFMLGKASFLSFKKGHPILFRGSQVKINKSNDNNYIVTVRLLRKEYAEELYNGITVKTKNKKEEKVHKRNINDMNIRFYIKANDKYNKVILERVLNKEYKIGGSRIFMKGNKIFFDLVYSFEQKKDEKLDKNRIMGIDIGYNIPAAVAINDMPYKKWFIGDRKEIEDFRTKIEVRKKQLQKWSVWAGDGRVGHGIKTRIKPVLNIGEKINNFKNLKNHVWSREIINIALKNKCGTIQMEKLEGIIPEEYSFLKNWSFYDLQQKIEYKAREHGIDVVYIDPAYTSARCSKCGHIHKSYEKKDWRPEQGQFICQVCGYKENADINAARNIATPNIEKIIKEQLEKQEREQRNQKYIS

SEQ ID NO: 244 - protein, 430 aa, synthetic construct
  REGION 1..430: note = TnpB homolog
MGTVTKVMKYELRYLDGSGSFHDMQNYVWQLQRQTREILNRTIQEATLWDYRSREHFLEAEEYLDVYAETGYKTLDGYIYNRLKGSYGDFAGANLNATLRKAWKKYKTSKTEVLRGTMSLPSYKGDQPLVLHNGSVKLQGDSRDAVVELTLFSNTFKKREGIKGNPSFSLLVRDNTQRSIYQSLIDGVYKLGECQLVYQKKKWFLLLTYTFEARQHEVDPEKILGVDLGEAYAIYASSKDNFGSLKIEGGEVTDYAKGLERRKRALQQQARYCGEGRVGHGTKTRVTEAYKAEDRLANFRKTINHRYSKALIDYAVKNGYGTIQMEDLSGIKADTGFPKRLQHWTYYDLQSKIEAKAKEYGIHVVKVDPSYTSQRCSKCGHIDSQNRKTQERFLCVSCGFSCNADFNASQNLSIKGIEKIIKKTKGAKVE

SEQ ID NO: 245 - protein, 431 aa, synthetic construct
  REGION 1..431: note = TnpB homolog
MSVKIASFSLIYKEDYNELNYDDLYNVLIQLQNESAKIANRAVQIYWENSNYCRQVKSMTGRFPTKDELLKHYGCSEQNYVYRLLTKEFYKNSTGNISTIIQFVGKRYKRYYPDYLSGKRSIESYKSSFPIYLCKNNIRVFKEDGKYYIKLGLISALYKSELSIHSGSVIFELGFGKSSSYKTLLDNIINQLFSLTSSKIIFLKKKIIIQLGYNTNSNIILDNSSCRVMGIDIGVAKPFVYAFNDITDFNFVDGNEIKNFQKQMLSRRQSLGRQTKNCADSKIGHGIHKRIEGIEKLGQKESNFRNRINHQYSRMIVDAAIKYKCTTIQIEDLSGISSENKFLKSWPYYDLQSKIEYKAKECGIDVVKINPKFTSQRCSKCGYISKENRKTQAGFKCKNCGFEENADLNAARNIAIPKIDSIIQESLRATT

SEQ ID NO: 246 - protein, 434 aa, synthetic construct
  REGION 1..434: note = TnpB homolog
MNKVVKLSLICEQTDKDGNKIEHGEVYKILWELQRQTREIKNKTIQYCWEYSNFSSDYYKINHEYPNEKEILSFTLKGFVNDKFKKGNDLYSGNCSTTTGNVCSEFKNSKSDFLKGEKSIINYKAYQPLDIHNKCILIEHTNNEFYVRLKLLNRPAIKKYNFANSEFNFKIIVKDNSTRTILERCIDKIYDVAASKLIYDKKKKMWVLNLVYAFDNKSEYVLDKNRILGVDLGIHYPICASVYGEWNRFTIDGGEIEKFRKTVEARKKSMLRQGKNCGDGRIGHGISARNKPVYKIEDKIAKFRDTANHKYSHALIQYAIKNNCGVIQMEDLTGITNEADRFLKNWSYYDLQTKIKYKAKEVGIDIVYIKPKYTSQRCSKCGYIDKENRNKQASFVCLKCGFKANADYNASQNISIKDIDKLIEEMYNSSANTE

SEQ ID NO: 247 - protein, 447 aa, synthetic construct
  REGION 1..447: note = TnpB homolog
MNKCIKVELKSCLEKNLSNKQSQKFLKDIQYLSWKGCNRAITYLYNHDMKNSELKYKNLPKIDPNKEYGKSLGSWIEDKLKEIMVGCLTTNVAQTRAFVMNRYKQDKKQGLLKGNVSLSNFKRNMPIIIHNKAYKIIKDDKGYIAEIGLFNLIKQKELGIKRLTFRINKLDGNKKSTLNKIINEDYKLGSGQIKQDSKGKWYLLISYSFKNEIVEGLDKDKILGIDLGIVNTVAMSIYNIKKDTWEQTRYKDTVIDGEELIHFRKKIEARKKSLSIGSKYCGDGRIGHGYKTRMKPFLNIKDKISKFRDTYNHKISRYIIDFAIKNKCGAIQMEDLSGFPEYQTEKFLKDWTYYDLQNKLKYKAEEIGIDIIFINPKYTSQRCSKCGNINNKNRDCKKDQAKFQCIICGYKENADINASKNISIPYIDDIIKEYLKENNSIKVDFPT

SEQ ID NO: 248 - protein, 431 aa, synthetic construct
  REGION 1..431: note = TnpB homolog
MPKQISKVMKYELKYLGEEDFYEMQKMLWSLQEDTREILNKTIQIFFHWDYTNKESLETTGKALNLVEETGYKDISGYVYDKLKSRYPDMSRGNLSATIRAASKKYRSSKVDILKGTMSIPSYKKDQPIILRPDGIRLHEREMIYTVELSLFSGDFKKKKAWKSNVLFQIKACDKAQKAIMQRLLSREYKLGESKLVYKKKKWFIYITYSFKKTDAKLDKNKILGVDLGVTYAIYACSIGEYGSFSIKGEEALEYAKRLEARTISKQKQARYCGEGRIGHGIKTRLSTVYSTRNKLANHRDTLNHRYSKAVVDYAVKNRYGTIQMENLSCIKKNTGFPKRLQHWTYYDLQSKIEYKAAEQGIQVIKINPKFTSLRCSQCGCIHKDNRKTQESFQCVECGYKDNADHNAALNISIPQIDLIIKEEMTSAKEK

SEQ ID NO: 249 - protein, 427 aa, synthetic construct
  REGION 1..427: note = TnpB homolog
MSKVMKYELKYLGEEDFYEMQKMLWSLQEDTREILNKTIQIFFHWDYTNKESLETTGKALNLVEETGYKDISGYVYDKLKSRYPDMSRGNLSATIRAASKKYRSSKVDILKGTMSIPSYKKDQPIILRPDGIRLHEREMIYTVELSLFSGDFKKKKAWKSNVLFQIKACDKAQKAIMQRLLSREYKLGESKLVYKKKKWFIYITYSFKKTDAKLDKNKILGVDLGVTYAIYACSIGEYGSFSIKGEEALEYAKRLEARTISKQKQARYCGEGRIGHGIKTRLSTVYSTRNKLANHRDTLNHRYSKAVVDYAVKNRYGTIQMENLSCIKKNTGFPKRLQHWTYYDLQSKIEYKAAEQGIQVIKINPKFTSLRCSQCGCIHKDNRKTQESFQCVECGYKDNADHNAALNISIPQIDLIIKEEMTSAKEK

SEQ ID NO: 250 - protein, 497 aa, synthetic construct
  REGION 1..497: note = TnpB homolog
MGESVKAIKLKILDMFLDPECTKQDDNWRKDLSTMSRFCAEAGNMCLRDLYNYFSMPKEDRISSKDLYNAMYHKTKLLHPELPGKVANQIVNHAKDVWKRNAKLIYRNQISMPTYKITTAPIRLQNNIYKLIKNKNKYIIDVQLYSKEYSKDSGKGTHRYFLVAVRDSSTRMIFDRIMSKDHIDSSKSYTQGQLQIKKDHQGKWYCIIPYTFPTHETVLDPDKVMGVDLGVAKAVYWAFNSSYKRGCIDGGEIEHFRKMIRARRVSIQNQIKHSGDARKGHGRKRALKPIETLSEKEKNFRDTINHRYANRIVEAAIKQGCGTIQIENLEGIADTTGSKFLKNWPYYDLQTKIVNKAKEHGITVVAINPQYTSQRCSMCGYIEKTNRSSQAVFECKQCGYGSRTICINCRHVQVSGDVCEECGGIVKKENVNADYNAAKNISTPYIDQIIMEKCLELGIPYRSITCKECGHIQASGNTCEVCGSTNILKPKKIRKAK

SEQ ID NO: 251 - protein, 464 aa, synthetic construct
  REGION 1..464: note = TnpB homolog
MVEQGVTITLNKSDKNTYTIARKVRLAVDGDKEEVNRVYQFLRDGIYNQNKAYNIFISSVYSAIINGASTEELNEIYKRGSRKPKEDDETYSLYKFGEIEFPVGVGTTASLKQMVKNDLKKAKNDGLFKGKISLPNRKLNAPLRIESACFSFIHNYNSYQEFLDHLYTDDCEIIMKFVNNIRFKVNLGQACKTHELRSVFQNIFEENYKVCGSSIEIDGTKIILNLSLTIPKKKHELDESIVVGVDLGIAVPAVCSLNNNTYIKKFIGSRNDFLRERTKLKAQRRNVQKSLKFTSGGHGRKKKLRHLEVFTEHEKNWVKNYNHRVSKEIVDFALSNDAKYINIENLQGFDSSNFLLANWSYYQLQQQIEYKADMHGIIVRKVNPYHTSQRCSCCGFESPDNRPKDKKGQAYFKCLNCGTEMNADFNASQNIARSTDFSIGEVTLEEDKKKHNKSKKIPKEKQAA

SEQ ID NO: 252 - protein, 433 aa, synthetic construct
  REGION 1..433: note = TnpB homolog
MKITKTMKYEIDKSIDVPWKTFLSVLRDVQYAVWKTGNIAVKMTWDFQQEAWSYRQRFGEQLKFSDLGTGNKSQSTDIYQRACSEYPNVASSVLDATIRMAQDRYKTDAPDIYDGLKTIPYFKRELPIPIRAQQTKLTRKGTKRYVSFALLSKEGAKKSELPTRYNVQIRTGKGAREIFDRLVDGEYKLCDSKILRKKGKWYLALSYSFEAENPQELDPKRVMGVDLGIVKTAYMAFNFDEYLRYEIEGGEISAFRGRIESRRKSLLKQARYCGEGRRGHGRKTRMKPLEKLRDKVANFRRTKNHHYSKYIVEMAAKHGCGTIQMEDLSGINKRDKFLANWSYYELQSFVKYKAKERGIKVVLVDPNYTSQRCSCCGYIAEGNRKTQETFKCVICGYKTNADFNAARNIAEPRIKALIDAELKRQEKERKEAM

SEQ ID NO: 253 - protein, 422 aa, synthetic construct
  REGION 1..422: note = TnpB homolog
MIKVYRYEIVKPLDLDWKEFGTILRQLQQETRFALNKATQLAWEWMGFSSDYKDNHGEYPKSKDILGYTNVHGYAYHTIKTKAYRLNSGNLSQTIKRATDRFKAYQKEILRGDMSIPSYKRDIPLDLIKENISVNRMNHGDYIASLSLLSNPAKQEMNVKRKISVIIIVRGAGKTIMDRILSGEYQVSASQIIHDDRKNKWYLNISYDFEPQTRVLDLNKIMGIDLGVAVAVYMAFQHTPARYKLEGGEIENFRRQVESRRISMLRQGKYAGGARGGHGRDKRIKPIEQLRDKIANFRDTTNHRYSRYIVDMAIKEGCGTIQMEDLTNIRDIGSRFLQNWTYYDLQQKIIYKAEEAGIKVIKIDPQYTSQRCSECGNIDSGNRIGQAIFKCRACGYEANADYNAARNIAIPNIDKIIAESIK

SEQ ID NO: 254 - protein, 428 aa, synthetic construct
  REGION 1..428: note = TnpB homolog
MKLVKTMRYQIIKPLSCDWDTLGTVLRELQRDTHSVLNKTIQLCWEWQGYSSEYKAANGTYPTPKDTLGRSLEGYVYDRLKVQFPKMYTPNLSQTIQRAMLKWSADSKAIFKGEVSIPSYKKDVPLDLRKDSIHIERRGHDYILSLGLVSRAYKKELGLPECQIEVLIGTPDKTQRVILARLLTGEYTVSGSQIVWDKRNRKWFVNLAYHFEARPEQLDKTKILGVDLGVVFPVYMAVADGHFRAGIPGGEIEEFRRRVEARRRQLLRQGKYCGDGRIGHGRATRTRPLDKIADKIARFRDTINHKYSRYVVETARKLGCGVIQMEDLTGIREENLFLANWPYHDLQRKIEYKAREYGIEVRYVRPQYTSQRCSDCGYIHPDNRPEQAKFRCLACGFETNADYNAARNIATEGIEELIAAALNKASVV

SEQ ID NO: 255 - protein, 471 aa, synthetic construct
  REGION 1..471: note = TnpB homolog
MPIITRKIELKIVKDGLTDEEYDQQWKYLYQINNTIYQAANRISTHCLFNDEYEMRLKLHMPRYKEIEKELKKLDSDKKTSDKEIRDRLLNERKELDEDVKNKKKDFLQCSKQNSTYQLVSKEFKQYIPSDILANLNQKIQENYNNNQKKIESGERALSTYKKGMEIPFSIRENKRLKLFIKEEGIYLKWFKEILFRLEFGKDASNNRCIVERLIESDRQQKNKGEDYVANNSSIKLVKNGKSTRIFLLLSIDIPAKKQVLDKEVVLGVDLGIKCPLYLAINKDDNFKMQIGNIEHFHNQRTMFQKRFKSLQKLMCTQGGHGRKKKLEPLEKLKEKERNWVHTQNHVYSREVIRQALKHNAGTIHMESLKDFGKGKDGYVKDEYKYLLRYWSYYELQSMIEYKAKLEGIEVKYIDPAYTSQTCSYCGERGERKKQEEFVCTNPQCKRCGEKINADFNAARNIAMSKKIVER

SEQ ID NO: 256 - protein, 389 aa, synthetic construct
  REGION 1..389: note = TnpB homolog
MWEYKKVEYKNKYGEYPNEKEMYGKTYRNVVESEMKLIMNTINTANVGQTNAFVMKKWNTDKRDIMNYKKSLANFKLNMPIYIKNSSYKIIKTPTGYEVDCAIFNKSLELKHLTFIIDKLDGNKKSTLNKLMDENYKQGAAQITRDNKGKWNLIISFSFETEKKELDPNRIVGIDVGITNALTMQIWDNNLQEWDRLSWRKCVLDGKELIHYRQKIEARRIALLKNSKVAEENTGKAGHGRTKRIEAISNMSEKVKHFRDTLNHKYSKYVVDFAVKNNCGCIQMENLSGFGENISETLLKNWSYFDLQQKIKYKADEDGIEVNFINPRYTSLRCSSCGNIDKENRDCKNNQAKFECIVCGHKENADINASKNISLPNIEEIIKEQLKTK

SEQ ID NO: 257 - protein, 417 aa, synthetic construct
  REGION 1..417: note = TnpB homolog
MPKQEEEGMIITRKIEIACRNKDQYPLLQDYLKQCRLMANKAMTNYYILWQEMLETKPKNQTQKDYFLKKHGCSFQNTGYRYLRRCFGGMPSYLRRDVANRVYQDFRADLKNGLLKGERSLRNYRTGHLPLHNKDIQLCKEETSSDYLLRWRMGIEFVLLFGRDRSGNRIIADRLIEGTYRVSGSQIYKDWRKKKWFVLLCVKIPQQDNNLDETAVVGVDLGLSTPAVCALSNGMARAYIGSSNLLKRFEMQKKQRSRQREFIPATNKHGRQKVVKAIYAMKDKERRFVHSFNHAISKKIIQFALKYKAAVIRMEDLSGYNGDETVLRNWSYYELQSMIEYKAEKEKIRVEKIPACYTSRACSQCGFIDKENRKTQAQFECVKCGFKENADYNAALNIARGGVKIPEENQEDFGENE

SEQ ID NO: 258 - protein, 471 aa, synthetic construct
  REGION 1..471: note = TnpB homolog
MPIITRKIELKIVKDGLTDEEYDQQWKYLYQINNTIYLAANRISTHCLFNDEYEMRLKLHMPRYKEIEKELKKLDSDKKTSDKEIRDRLLNERKELDEDVKNKKKDFLQCSKQNSTYQLVSKEFKQYIPSDILANLNQKIQENYNNNQKKIESGERALSTYKKGMEIPFSIRENKRLKLFIKEEGIYLKWFKEILFRLEFGKDASNNRCIVERLIESDRQQKNKGEDYVANNSSIKLVKYGKSTRIFLLLSIDIPAKKQVLDKDVVLGVDLGIKCPLYLAINKNDNFKMQIGDIEHFHNQRTMFQKRFKSLQKLMCTQGGHGRKKKLEPLEKLKEKERNWVHTQNHVYSREVIKQALKQNAGTIHMESLKDFGKGKDGYVKDEYKYLLRYWSYYELQSMIEYKAKLEGIEVKYIDPAYTSQTCSYCGERGERKKQEEFVCTNPQCKRRGEKINADFNAARNIAMSKKIVER

SEQ ID NO: 259 - protein, 422 aa, synthetic construct
  REGION 1..422: note = TnpB homolog
MKYELTYLDGCGDFHNMQNELWALQRQTRELLNRTVQIAYHWDYKGSEHYRETGQPMDVYTETGYKRLDGYIYSCLKDDADSFSAANVNATIQKAWKKYKSSKSDIMQGKMSLPSYKRDQPLILYARNVKISNEQRNPAVQFTLFSKSYKEEKGYSDVQFVMHLNDATQKAIFQKIASKEYGLGECQLVYSKPKWFLLLTYNFTPEDRRLDPDRILGVDMGETFALYASSKDEYGSLKIEGGEVREFAKRMEARKRSMQRQSAHCGEGRIGHGTKTRVSDVYKAEDKIANFRSTVNHRYSKKLIEYAVQHQYGTIQMEDLSGIRESTGFPKFLRHWTFYDLQQKIEAKAREQGIRVVKVDPSYTSQRCSKCGNIDKANRPTQAQFCCSKCGYKTNADFNASQNLSIRGIDRIIKETLGANPK

SEQ ID NO: 260 - protein, 432 aa, synthetic construct
  REGION 1..432: note = TnpB homolog
MSKGSLAKVMKYELRYLDGAGSFEQMQERLWVLQRQTREILNRSTQISFHWDYTSREHFEQTGQYLDVFSETGYKRLDGYIYSRVKDSCGDMASGNINATLQKAWNKYGTSKLDVLRGQMSLPSYKKDQPLVIEKHNIRLSMDGQQALAEITLFSNKFKKENSLSSNVRFAFQLHDGTQRRILNSVLSGEYGLGQCQLVYDRPKWFLLLTYTFTPQNRQLDPDRILGVDLGECYALCASVFGEYGSLRIEGGEVTAYAKKLEARKRSLQKQAAVCGEGRKGHGTKTRVADAYQMQDRIANFRDTVNHRYSKALIDYALKNQCGTIQMEDLSGIRQDTGFPKFLQHWTYYDLQSKIENKAKEHDIRIVKINPRYTSQRCSKCGAIDSGSRTSQARFCCTKCGFTANADYNASQNISIKGIDLLIEKELGAKAE

SEQ ID NO: 261 - protein, 471 aa, synthetic construct
  REGION 1..471: note = TnpB homolog
MATKEKRIVKVMRLRILKPAGEMSWSQLGKLLRDTRYRVFRLANLAVSEAYLNFHLWRTGRSQEFKADDMGKLSRRLRQMLADEGVAADELDRFSPTGAVPDAVSGPLFQYKIRAITNKNKWREVIRGTASLPTFRLDMAIPVRCDKARMRRLERMENGDVQVELTICRKPYPRVVLQTGDIGGGQEAILARLLDNTGNDLTGYRQRVFEIKQERQTSKWWLYITYDLPAPQTGKADPDVVVGVDVGYAVPLYVAINNGHARLGWRQFDALGRRIRKLQTQVLARRRSIQRGGRVNISHATARSGHGVKRKLLPTEILQRRIDKAYQTLNHQLSASVIDFARDHGAGVIQVEDLEGLKEELTGTYIGARWRYHQLHQFLKYKAEENGIEFRAVNPRFTSRRCSKCGHINVAFDRAYRDAHRENGKTARFICPQCGFEADADYNAARNLATLDIEALIEAQCARQGLTKDAL

SEQ ID NO: 262 - protein, 468 aa, synthetic construct
  REGION 1..468: note = TnpB homolog
MPTITRKIELNLCTEGLADEEQKAQWNLLYHINDNLYKAANNISSKLYLDDHVSSMVMLKHAEYLTLVRALEKAQKQKTPDETVIEDLRRQVAAAEKDMTDQELAICNYATEMSTQSLSYRFATEIETNIFAQILDCLKQGVYATFNSDAKDVKRGERAIRNYKKGMPIPFPWNKSLKIEHKDGEFYLLWYNGLRFHLNFGKDRSNNRLIVQRCMKMDKDYEGDYKMCNSSIQFVKREGKPKFFLLLVVNIPQEHVELDKKIVVGVDLGINSPAYVATNVTMERQQIGRRETFLNGRMSFQRRYKSLQRLQTTAGGRGRKKKLEPLERLRNAEHNWVHTQNHLFSREVVQFAVKARAATIHMEDLSGFGKDNDGNADERKEFVLRNWSYYELQTMISYKAQKYGIKVEKIRPAYTSRTCSWCGHEGFRKGEIFICENPACEKCGEKENADYNAARNIANSKDIIKNHG

SEQ ID NO: 263 - protein, 384 aa, synthetic construct
  REGION 1..384: note = TnpB homolog
MSFYEALMNDTNVELFMKFCNNITFKFCLGNVKDSLYLRRTLESLFNGEIKACDSSIQVEGKKIMLNMCVDYPKRTYELNKNIVMGIDIGFIVPIMCALSNHEYKRLALGSREFINHHRIMYQKQRSSVSKSMRDNSTNGHGRNKKVRPVDEIKANESNFAKTYSKTLARKAVDYAIKNHVGVIQMENLKHISRDERQQFVLRNWGYYELQKSIEYAAEQAGIEVRYVEPAYTSQVCSICGHRGERTAQATFVCTNPDCKIHGKYKEAEKTDFDVNADFNGARNIAMSDHFVTDGTKSVELVFNEEFTNEQREIFANCVSENQTYTHCYVAGNTVSIMCDDGYWHDFDLKIVEKAVNDDSVDKLNGEKKEKKAKTTKTKKEKAA

SEQ ID NO: 264 - protein, 496 aa, synthetic construct
  REGION 1..496: note = TnpB homolog
MPTITRKIELKIVKDRLTDEKERLTDEKYDQQWKYLYQINNTIYQAANRISTHCLFNDEYEMRLKLHMPRYKDIEKKLEEIEKKQKGLNTKKKTSDKEKRDRLINEQRQLVDERNELDEDVKNKKKDFFQCSKQNSTYQLASKEFLKYIPAEILTDLNRYVQNNHNNNKKKVKSGERALSTYKKGMGIPFSIKPQSGLRLFVKEEGIYLKWFKGILFRLEFGKDTSNNRCIVERLIESDKQQKKNKGEDYVANNSSIKLIKKGNDKSTRIFLLLSIDIPAKKQVLDKEVVLGVDLGIKCPLYLAINKNDNFKMQIGDIEHFHNQRTMFQKRFKSLQKLMCTQGGHGRKKKLEPLEKLKEKERNWVHTQNHVYSREVIKQALKQNAGTIHMESLKDFGKGKDGYVKDEYKYLLRYWSYYELQSMIEYKAKLEGIEVKYIDPAYTSQTCSYCGERGERKKQEEFVCTNPQCKRRGEKINADFNAARNIAMSKKIVKDN

SEQ ID NO: 265 - protein, 421 aa, synthetic construct
  REGION 1..421: note = TnpB homolog
MDKTLRDIQYVTCKASNKAMQMYYMWEYEKLEYKNKYGEYPNEKEMYGKTYRNVVEAEVKAIMNTINTSNTGQTNAFVMKKWNTDKKDIMNYRKSVASYKLNMPIYLKNSSYKILQGESGYEIDCAIFNKSQGLKHLTFTIDKLDGTKKATLNKLIESKNLSELINGAYKQGAMQIVKKKNKWCMLISFGFEAVKRELDTNRIVGVDVGIVNALTFQVWDNTTQKWDRLSWRDCLLDGKELIHYRQKIMARRIALLKNSKLSDENKGKAGHGRVKRIGPINTISDKVKAFRDTLNHKYSKYVIDFAIKNNCGCIQMEDLSGYSESVSETFLKNWSYFDLQSKIKYKAEENGLAINFIKPYHTSLRCSLCGNIQKENRDCRNNQSRFKCTVCGYEENADINAAKNISLPNIEQLIKEQLKIK

SEQ ID NO: 266 - protein, 478 aa, synthetic construct
  REGION 1..478: note = TnpB homolog
MPILTRTIELIPIGDKEERDRCYKWIRDFMEEQSKMMNQYMSALYIAAVEEVSKDDRKELNNLYNRIATSKKGSAFSKEECNLPKGLGANYGQRVRSDFDTACENGLLHGRVSLPTYKKNFPIILAPIYVNLQKNNIEEKGKSAGFYHNYASYNELYDALKEENKPEIIWNFVQKMQYQIKFGNPYKSAFLRDEILHFLEGEYKAVGSQLSINSRGKIILNLSLDVPQKKVKLDENIVVGIDIGLAVPVMCAINNDYYKRLAVGDFEAFTRMREKLYSQKCKLQRQLKYTSGGHGRKKKLASLNAIRDREHRFVHTMNHKYSSEVINFALKNNAKYINMEDLTGFGKDNKGNAIDDYQFVLRNWSYFELQKMIQDKAQKYGIVVRKVESAYTSQLCSCCGEMGERVSQSVFRCLNPNCISHNKYEKQRKSGVGNYHFNADFNAARNISMSTNYTKKKRKTKAEKVEERKKNAIEKTAG

SEQ ID NO: 267 - protein, 424 aa, synthetic construct
  REGION 1..424: note = TnpB homolog
MKKTVRLQIVKPMDEDWEILGRVLHDIRYQTRQVLNKTIQLCWEYSNFSSEYKALHGDYPKNKEILHYTSMHGYAYNQLKEQYYYIQSGNCSQTVKRAVDKWKSDLKEILRGDRSIPSYKKDIPIDIVKDAVSLEHDEKNGNYIATLSLMSTAYRKEMERKSGQFRVLLHSGDNSKKTILKRLVQGEYQHTASQIVKKGKKWFLNLSYKFDVLQTPFQTERVMGVDMGVIYPIYMAFNYHDHLRYKIQGGEIERFRRQVESRKKALQDQGKYAGSGRVGHGTKTRIDPLEVIRDKIANFRETKNHHYSRYVVDMAEKHECATIQLEELKGIHQDDAFLKRWSYHDLQEKITYKAEEKGIQVIKVDPQKTSQRCHHCGNIDSNNRKEQASFLCTSCGMETNADFNAAKNISIPGIEQIIQTEMKS

SEQ ID NO: 268 - protein, 455 aa, synthetic construct
  REGION 1..455: note = TnpB homolog
MKMTKVVKLALISNVTDKDGNKVEYNELNRCLWDLQKETRDLKNAVVRECWEWYGFTNDYYKLNEEYPNERDYLKKAKSDGTIKDYALDGFIYAKYSKKYNLHSGNYSQTLRDACGSFKNNLKEILRGDKSILSYRADQPLDIKKTCIGLEYDKDTNTYYVTLVLLNKNGVKHYNISDFRFKITVKDNSTRTILERCFDGVYGISASKLIWNRKKSQWFLNLCYSFDKVEVKELDKKKILGVNLGVYYPLYASISGEKDRLAISGDEIIEFRKRIEARRTALKKQAAVCGDGRIGHGYKTRMKPLQNVSDKIANFRDTFNHKASKKLIDFAIKNDCGIIQLENLKGVTKNSEGFLKNWSFYDLQSKIENKAKERGIKVVYIEPAYTSLRCSKCGCIHKDNHPTREQFICQECGYRVLHDYNASQNIAVKDIDKIIKAELEKTEPEKKTEEEKPEK

SEQ ID NO: 269 - protein, 453 aa, synthetic construct
  REGION 1..453: note = TnpB homolog
MTKVVKLALISNVTDKDGNKVEYNELNRCLWDLQKETRDLKNAVVRECWEWYGFTNDYYKLNEEYPNERDYLKKAKSDGTIKDYALDGFIYAKYSKKYNLHSGNYSQTLRDACGSFKNNLKEILRGDKSILSYRADQPLDIKKTCIGLEYDKDTNTYYVTLVLLNKNGVKHYNISDFRFKITVKDNSTRTILERCFDGVYGISASKLIWNRKKSQWFLNLCYSFDKVEVKELDKKKILGVNLGVYYPLYASISGEKDRLAISGDEIIEFRKRIEARRTALKKQAAVCGDGRIGHGYKTRMKPLQNVSDKIANFRDTFNHKASKKLIDFAIKNDCGIIQLENLKGVTKNSEGFLKNWSFYDLQSKIENKAKERGIKVVYIEPAYTSLRCSKCGCIHKDNHPTREQFICQECGYRVLHDYNASQNIAVKDIDKIIKAELEKTEPEKKTEEEKPEK

SEQ ID NO: 270 - protein, 450 aa, synthetic construct
  REGION 1..450: note = TnpB homolog
MSTVVKVMKYQIICPVNIEWKAFETYLRTLSYQVRTIGNRTIQKLWDFDNQSLNHFRENGVYPSAQQLYGCTQKTISGYIYDQLKEEYQDMNKANMSTTLQKTIKTWNSRKKEIRSGEMSIPSFRNNLPIDIHGNSIQITKEKSGDYIASLSLFSSNFIIENNLPNGKIQVKLSTRKQNSMKVILDRIIENTYAKGACMLHKHKNKWYLSIIYKPTVKEEHKFEEDLVMGIDMGKINVLYFAFNKGWIRGAISGEEIEAFRKKIEHRRISLLRQGKYCSGNRVGKGREKRIKPIDVLNNKIAKFRNATNHKYANYIVQQCLKYNCGTIQLENLQGISKEQTFLKNWTYFDLQEKIKQQAHQYGMKVVTIDPSYTSKRCSECGYIHKNNRKSQSTFECQQCNLKVHADYNAAKNISIYNIEKVIQKQLKLQEKLNSKKFTEQYIEQVENIN

SEQ ID NO: 271 - protein, 522 aa, synthetic construct
  REGION 1..522: note = TnpB homolog
MDNTITITRKYALIPEFSDRKEWKKRVYDFTINDLEQKIDYRNKKKQDTSKLESQLEYIKNGGDFTRSMVNNYTYSLVSTAMEEEARRKNYILSWIFSEMRANRVDQMESLKDKFKFVSDTINYAYRKAGSNKGSLFDETEIRCILKSYGIAFSQELTKEIKELVKNGVLEGKVVIPTYKLDSPFTIAKSHFSFEHDYDSFEELCEHISDSDCKMYMNYGGDNKKDGINPASIARFRISLGHGKNKDELRATLLKVYSGEYQYCGSSIQITKNKIILNLTMKIPKIETKLDKNTVVGVDLGIAVPAMCALNNNMYERLAIGSADEFLRVRTKYQAQRRRLQKSLKNSSAGHGRKKKLKALDRMDKAESHFVETYCHIVSKRVVEFAVKNRAKYINIENLNGYDTSQFILRNWSYYKLQQYITYKAERYGIAVRKINPCYTSQVCSVCGNWEDGQRKTQASFKCANQKCESHKKYKYGFNADFNAARNIAMSTLFMEDGEVTEKKKEEAREYYGIKKENSKAV

SEQ ID NO: 272 - protein, 453 aa, synthetic construct
  REGION 1..453: note = TnpB homolog
MKYLSTVVKVMKYQIICPVNIEWKAFETYLRTLSYQVRTIGNRTIQKLWDFDNQSLNHFRENGVYPSAQQLYGCTQKTISGYIYDQLKEEYQDMNKANMSTTLQKTIKTWNSRKKEIRSGEMSIPSFRNNLPIDIHGNSIQITKEKSGDYIASLSLFSSNFIIENNLPNGKIQVKLSTRKQNSMKVILDRIIENTYAKGACMLHKHKNKWYLSIIYKPTVKEEHKFEEDLVMGIDMGKINVLYFAFNKGWIRGAISGEEIEAFRKKIEHRRISLLRQGKYCSGNRVGKGREKRIKPIDVLNNKIAKFRNATNHKYANYIVQQCLKYNCGTIQLENLQGISKEQTFLKNWTYFDLQEKIKQQAHQYGMKVVTIDPSYTSKRCSECGYIHKNNRKSQSTFECQQCNLKVHADYNAAKNISIYNIEKVIQKQLKLQEKLNSKKFTEQYIEQVENIN

SEQ ID NO: 273 - protein, 453 aa, synthetic construct
  REGION 1..453: note = TnpB homolog
MTYLSIAVKVMKYQIVCPVNVEWKVFETYLRTLSYQSRTIGNRTIQKIWEFDNLSLNHFKETGEYPSAQHLYGCTQKTISGYIYDQLKEEYQDINKANMSTTIQKTLKNWNSRKKEIWRGEMSIPSFRNNLPIDIHGNSIQIIKEKSGDYIASVSLFSSKFIKENDLPNGKILVKLSTRKQNSMKVILDKIVNSIYAKGACMLHKHKNKWYLSITYKATIKEEHKFDEELIMGIDMGKINVLYFAYNKGLVRGAISGEEIEAFRKKIEYRRISLLRQGKYCSENRIGKGRKKRIKPIDVLNDKVAKFRNATNHKYANYIVQQCLKYNCGTIQLEDLQGISKEQTFLKNWTYFDLQEKIKNQANQYGIKVVKIDPSYTSQRCSECGYIHKKNRQDQSTFECQQCSFKIHADYNAAKNISVYNIEKVIQKQLELQEKLNLTKYKEQYIEQMENIN

SEQ ID NO: 274 - protein, 450 aa, synthetic construct
  REGION 1..450: note = TnpB homolog
MSIAVKVMKYQIVCPVNVEWKVFETYLRTLSYQSRTIGNRTIQKIWEFDNLSLNHFKETGEYPSAQHLYGCTQKTISGYIYDQLKEEYQDINKANMSTTIQKTLKNWNSRKKEIWRGEMSIPSFRNNLPIDIHGNSIQIIKEKSGDYIASVSLFSSKFIKENDLPNGKILVKLSTRKQNSMKVILDKIVNSIYAKGACMLHKHKNKWYLSITYKATIKEEHKFDEELIMGIDMGKINVLYFAYNKGLVRGAISGEEIEAFRKKIEYRRISLLRQGKYCSENRIGKGRKKRIKPIDVLNDKVAKFRNATNHKYANYIVQQCLKYNCGTIQLEDLQGISKEQTFLKNWTYFDLQEKIKNQANQYGIKVVKIDPSYTSQRCSECGYIHKKNRQDQSTFECQQCSFKIHADYNAAKNISVYNIEKVIQKQLELQEKLNLTKYKEQYIEQMENIN

SEQ ID NO: 275 - protein, 497 aa, synthetic construct
  REGION 1..497: note = TnpB homolog
MPTITRKIELKIVKDRLTDEKERLTDEEYDQQWKYLYQINNTIYQAANRISTHCLFNDEYEMRLRLSYKSRYDKINKGLENIKTELEKLNTKKKTSDKEKRDRLINEQRQLVDERNELDEDVKNKKKDFFQCSKQNSTYQLASKEFLKYIPAEILTDLNRYVQNNHNNNKKKVKSGERALSTYKKGMGIPFSIKPQSGLRLFVKEEGIYLKWFKGILFRLEFGKDTSNNRCIVERLIESDKQQKKNKGEDYVANNSSIKLIKKGNDKSTRIFLLLSIDIPAKKQVLDKEVVLGVDLGIKCPLYLAINKNDNFKMQIGDIEHFHNQRTMFQKRFKSLQKLMCTQGGHGRKKKLEPLEKLKEKERNWVHTQNHVYSREVIKQALKHNAGTIHMESLKDFGKGKEGYVKDEYKYLLRYWSYYELQSMIEYKAKLEGIEVKYIDPAYTSQTCSYCGERGERKKQEEFVCTNPQCKRRGEKINADFNAARNIAMSKKIVKDN

SEQ ID NO: 276 - protein, 450 aa, synthetic construct
  REGION 1..450: note = TnpB homolog
MSTVVKVMKYQIVCPVNIEWKAFETYLRTLSYQVRTIGNRTIQKLWDFDNQSLNHFRENGVYPSAQQLYGCTQKTISGYIYDQLKEEYQDINKANMSTTLQKTIKTWNSRKKEIRSGEMSIPSFRNNLPIDIHGNSIQITKEKSGDYIASLSLFSSNFIKENNLPNGKIQVKLSTRKQNSMKVILDRIIENTYAKGACMLHKHKNKWYLSIIYKPTVKEEHKFEEDLVMGIDMGKINVLYFAFNKGWIRGAISGEEIEAFRKKIEHRRISLLRQGKYCSGNRVGKGREKRIKPIDVLNNKVARFRNATNHKYANYIVQQCLKYNCGTIQLENLQGISKEQTFLKNWTYFDLQEKIKQQAHQYGIKVVTIDPSYTSQRCSECGYIHKNNRQSQSTFECQQCNLKVHADYNAAKNISIYNIEKVIQKQLKLQEKLNSKKFTEQYIEQIENIN

SEQ ID NO: 277 - protein, 453 aa, synthetic construct
  REGION 1..453: note = TnpB homolog
MTYLSTVVKVMKYQIVCPVNIEWKAFETYLRTLSYQVRTIGNRTIQKLWDFDNQSLNHFRENGVYPSAQQLYGCTQKTISGYIYDQLKEEYQDINKANMSTTLQKTIKTWNSRKKEIRSGEMSIPSFRNNLPIDIHGNSIQITKEKSGDYIASLSLFSSNFIKENNLPNGKIQVKLSTRKQNSMKVILDRIIENTYAKGACMLHKHKNKWYLSIIYKPTVKEEHKFEEDLVMGIDMGKINVLYFAFNKGWIRGAISGEEIEAFRKKIEHRRISLLRQGKYCSGNRVGKGREKRIKPIDVLNNKVARFRNATNHKYANYIVQQCLKYNCGTIQLENLQGISKEQTFLKNWTYFDLQEKIKQQAHQYGIKVVTIDPSYTSQRCSECGYIHKNNRQSQSTFECQQCNLKVHADYNAAKNISIYNIEKVIQKQLKLQEKLNSKKFTEQYIEQIENIN

SEQ ID NO: 278 - protein, 453 aa, synthetic construct
  REGION 1..453: note = TnpB homolog
MMYLSKVVKVMKYQIVCPLNIEWKVFEIYLRTLSYHFRTIGNRTIQKLWEYDNQSLKHFKDTGQYPSVQQLYGCTQKTVSGYIYDQLKEEYQDINKANMSTTLQKTIKTWNSRKKEIWSGEMSIPSFRNNLPIDVHGNSVQVTKEKSGDYIASVSLFSSKFIKENDLPNGKILVKLSTRKQNSMKVILDKIIDSTYAKGACMIHKHKNKWYLSITYKATKKEGHKFDEDLIMGIDMGKINALYFAYNKGLVRGVISGEEIEAFRKKVEYRRISLLRQGKYCSENRIGKGRKKRIKPIEVLNDKVAKFRNATNHKYANYIVQQCLKYNCGTIQLEDLQGISKEQTFLKNWTYFDLQEKIKNQANQYGVKVVKIDPSYTSQRCSECGYIHKNNRQEQSTFECQQCSFKAHADYNAAKNISIYNIEKLIQKQLDLQEKLNLTKYKEQYIEQMENIN

SEQ ID NO: 279 - protein, 450 aa, synthetic construct
  REGION 1..450: note = TnpB homolog
MSKVVKVMKYQIVCPLNIEWKVFEIYLRTLSYHFRTIGNRTIQKLWEYDNQSLKHFKDTGQYPSVQQLYGCTQKTVSGYIYDQLKEEYQDINKANMSTTLQKTIKTWNSRKKEIWSGEMSIPSFRNNLPIDVHGNSVQVTKEKSGDYIASVSLFSSKFIKENDLPNGKILVKLSTRKQNSMKVILDKIIDSTYAKGACMIHKHKNKWYLSITYKATKKEGHKFDEDLIMGIDMGKINALYFAYNKGLVRGVISGEEIEAFRKKVEYRRISLLRQGKYCSENRIGKGRKKRIKPIEVLNDKVAKFRNATNHKYANYIVQQCLKYNCGTIQLEDLQGISKEQTFLKNWTYFDLQEKIKNQANQYGVKVVKIDPSYTSQRCSECGYIHKNNRQEQSTFECQQCSFKAHADYNAAKNISIYNIEKLIQKQLDLQEKLNLTKYKEQYIEQMENIN

SEQ ID NO: 280 - protein, 453 aa, synthetic construct
  REGION 1..453: note = TnpB homolog
MTYLSIAVKVMKYQIVCPVNVEWKAFETYLRTLSYQSRTIGNRTIQKIWEFDNLSLNHFKETGEYPSAQQLYGCTQKTISGYIYDQLREEYQDINKANMSTTIQKTLKNWNSRKKEIWRGEMSIPSFRSDLPIDIHGNSIQLIKEKSGDYIASVSLFSSKFIKENDLPNGKILVKLSTRKQNSMKVILDRLINSTYSKGACMLHKHKNKWYLSITYKATKKEGHKFDEELIMGIDMGKINALYFAYNKGLVRGVISGEEIEAFRKKIEYRRISLLRQGKYCSENRIGKGRKKRIKPIEVLNDKIAKFRNATNHKYANYIVQQCLKYNCGTIQLEDLQGISKEQAFLKNWTYFDLQEKIKNQANQYGIKVVKIDPSYTSQRCSECGYIHKNNRQDQSTFECQQCSFKVHADYNAAKNISVYNIEKVIQKQLELQEKLNLTKYKERYIEQMENIN

SEQ ID NO: 281 - protein, 450 aa, synthetic construct
  REGION 1..450: note = TnpB homolog
MSIAVKVMKYQIVCPVNVEWKAFETYLRTLSYQSRTIGNRTIQKIWEFDNLSLNHFKETGEYPSAQQLYGCTQKTISGYIYDQLREEYQDINKANMSTTIQKTLKNWNSRKKEIWRGEMSIPSFRSDLPIDIHGNSIQLIKEKSGDYIASVSLFSSKFIKENDLPNGKILVKLSTRKQNSMKVILDRLINSTYSKGACMLHKHKNKWYLSITYKATKKEGHKFDEELIMGIDMGKINALYFAYNKGLVRGVISGEEIEAFRKKIEYRRISLLRQGKYCSENRIGKGRKKRIKPIEVLNDKIAKFRNATNHKYANYIVQQCLKYNCGTIQLEDLQGISKEQAFLKNWTYFDLQEKIKNQANQYGIKVVKIDPSYTSQRCSECGYIHKNNRQDQSTFECQQCSFKVHADYNAAKNISVYNIEKVIQKQLELQEKLNLTKYKERYIEQMENIN

SEQ ID NO: 282 - protein, 453 aa, synthetic construct
  REGION 1..453: note = TnpB homolog
MTKVVKLALISNVTDKDGNKVEYNELNRCLWDLQKETRDLKNAVVRECWEWYGFTNDYYKLNEEYPNERDYLKKVKSDGTIKDYALDGFIYAKYSKKYNLHSGNYSQTLRDACGSFKNNLKEILRGDKSILSYRADQPLDIKKTCIGLEYDKDTNTYYVTLVLLNKNGVKHYNISDFRFKITVKDNSTRMILERCFDGVYGISASKLIWNRKKSQWFLNLCYSFDKAEVKELDKKKILGVNLGVYYPLCASISGEKDRLAISGDEIIEFRKRIEARRTALKKQAAVCGDGRIGHGYKTRMKPLQNVSDKIANFRDTFNHKASKKLIDFAIKNDCGIIQLENLKGVTKNSEGFLKNWSFYDLQSKIENKAKERGIKVVYIEPAYTSLRCSKCGCIHKDNHPTREQFICQECGYRVLHDYNASQNIAVKDIDKIIKAELEKTEPEKKTEEEMPEK

SEQ ID NO: 283 - protein, 450 aa, synthetic construct
  REGION 1..450: note = TnpB homolog
MSIAVKVMKYQIVCPVNIEWKTFEIYLRTLSYHFRTIGNRTIQKLWEYDNQSLKHFKDTGQYPSAQQLYGCTQKTISGYIYDQLKEEYQDINKANMSTTLQKTIKTWNSRKKEIWSGEMSIPSFRNNLPIDIHGNSIQIIKEKSGDYIASVSLFSSKFIKENDLPKGKILVKLSTRKQNSMKVILDRIIDSTYAKGACMLHKHKKKWYLSITYKSNIKEELKVDEDLIMGIDMGKINVLYFAFNKGLVRGAISGEEIEAFRKKIEHRRISLLRQGKYCSGNRIGKGRKKRIKPIEVLNDKIAKFRTATNHKYANCIVQQCLKYNCGTIQLEDLQGISKEQTFLKNWTYFDLQEKIKNQANQYGIKVVKIDPSYTSQRCSECGYIHKNNRQNQSTFECQQCSFKVHADYNAAKNISVYNIEKVIQRQLKLQEKLNLTKYKEQYIEQMENIN

SEQ ID NO: 284 - protein, 424 aa, synthetic construct
  REGION 1..424: note = TnpB homolog
MILTRKIQIIPLGEKEEIDRVYKYLRDGIFYQNKAMNQYMSALYIAAIKDISKEDRKELNRLYSRVSNSKKGSAYDKSIEFAKNMNLGYVVKQVKQDFANSCKNGLLCGKVSLPTYRKNNPLLVHVNFVRLRSTNYHQDNGMYHNYESHTDFLDHLYSKDLEVFIKFANNITFKMIFGNPHKSAYLRSEIQQIFEENYKVCGSSIQIDGKKIILNLSMDIPKQELELDENIVVGVDLGLAIPAMCGLNTNDYIRQSIGSKDDFLRIRTQLQSQRRRLQKSLASTSGGHGRQKKLKPLEKLKDRERNFVKTYNHYVSKNVVDFAVKNKAKYINVEDLSGFDSNQFILRNWSFYELQQFITYKAAKYGIEVRKINPYHTSQICSCCGHWEEGQRIDQAHFKCKSCGAELNADFNASRNIAMSTDFV

SEQ ID NO: 285 - protein, 492 aa, synthetic construct
  REGION 1..492: note = TnpB homolog
MPTITRKIELKIVKDRLTDEKERLTDEKYDQQWKYLYQINNTIYQAANRISTHCLFNDEYEMRLKLHMPRYKDIEKKLEEIEKKQKGLNTKKKASDKEERDRLLNEKQQLVNERKEIDEDVKNKKKDFLQCSKQNSTYQLVSKEFKQYIPSDILANLNQKIQENYNNNQKKIESGERALSTYKKGMEIPFSIRENKRLKLFIKEEGIYLKWFKEILFRLEFGKDASNNRCIVERLIESDKQQKGKGEDYVANNSSIKLVKNGKNTRIFLLLSIDIPAKKQVLDKEVVLGVDLGIKCPLYLAINKNDNFKMQIGDIEHFHNQRTMFQKRFKSLQKLICTQGAHGRKKKLEPLEKLKEKERNWVHTQNHVYSREVIKQALKQNAGTIHMESLKDFGKGKDGYVKDEYKYLLRYWSYYELQSMIEYKAKLEGIEVKYIDPAYTSQTCSYCGERGERKKQEEFICTNPQCKRRGEKINADFNAARNIAMSKKIVER

SEQ ID NO: 286 - protein, 453 aa, synthetic construct
  REGION 1..453: note = TnpB homolog
MTYLSIAVKVMKYQIVCPVNVEWKAFETYLRTLSYQSRTIGNRTIQKIWEFDNLSLNHFKETGEYPSAQQLYGCTQKTISGYIYNQLREEYQDINKANMSTTIQKSLKNWNSRKKEIWRGEMSIPSFRSDLPIDIHGNSIQLIKEKSGDYFANVSLFSSKFIKENDLPNGKILVKLSTRKQNSMKVILDRLINSTYSKGACMLHKHKNKWYLSITYKATKKEGHKFDEELIMGIDMGKINVLYFAYNKGLVRGAISGEEIEAFRKKIEYRRISLLRQGKYCSENRIGKGRKKRIKPIEVLNDKITKFRNATNHKYANYIVQQCLKYNCGTIQLEDLQGISKEQTFLKNWTYFDLQEKIKNQANQYGIKVVKIDPSYTSQRCSECGYIHKNNRQDQSTFECQHCSFKVHADYNAAKNISIYNIEKVIQKQLELQEKLNLTKYKEQYIEQMENIN

SEQ ID NO: 287 - protein, 450 aa, synthetic construct
  REGION 1..450: note = TnpB homolog
MSIAVKVMKYQIVCPVNVEWKAFETYLRTLSYQSRTIGNRTIQKIWEFDNLSLNHFKETGEYPSAQQLYGCTQKTISGYIYNQLREEYQDINKANMSTTIQKSLKNWNSRKKEIWRGEMSIPSFRSDLPIDIHGNSIQLIKEKSGDYFANVSLFSSKFIKENDLPNGKILVKLSTRKQNSMKVILDRLINSTYSKGACMLHKHKNKWYLSITYKATKKEGHKFDEELIMGIDMGKINVLYFAYNKGLVRGAISGEEIEAFRKKIEYRRISLLRQGKYCSENRIGKGRKKRIKPIEVLNDKITKFRNATNHKYANYIVQQCLKYNCGTIQLEDLQGISKEQTFLKNWTYFDLQEKIKNQANQYGIKVVKIDPSYTSQRCSECGYIHKNNRQDQSTFECQHCSFKVHADYNAAKNISIYNIEKVIQKQLELQEKLNLTKYKEQYIEQMENIN

SEQ ID NO: 288 - protein, 430 aa, synthetic construct
  REGION 1..430: note = TnpB homolog
MKEIAKVVKLELGWVFTDDGERAFPYSDLFEIQRQVALVKNKTIQLCWEWNNFGADFHAMSGAYPKTGDVTGYKTLDGYVYQRLKDDFSRMFKKNLNASVRSAQKAFETAKKSLHKGERSILSYRKDAPIELHNSAVSFSQEGRKYKAAVKVFSLSYAKEKGYAGTGVEFELSHLQGSPKEIVQRCMSGEYKIGESKLIWNEKKKKWFLYLTYKFTPAAVALDPEKIMGVDLGIACVAYMGFRFCEDRHVIPGHEVEHFRRRVEARKVELQRQGKFCGEGRIGHGRATRTKPVDQIGHAIARFRDTANHKYSRFIVDMAVKHGCGVIQMEDLHVHAEDKLLKDWTYFDLRTKLEYKAKEKGIEVRFVNPRYTSQRCSCCGYIEKENRKTQKEFICLECGFAANADYNAALNLATAGIEQIIDEYVSANHK

SEQ ID NO: 289 - protein, 450 aa, synthetic construct
  REGION 1..450: note = TnpB homolog
MSKNTYTITRKIQLIPVGDKEEVNRVYTYLRDGMKAQNMALNQYISALYFAMQNDATKDSRKELRNLFSRISTSKKGSAYDDTIEFAKGLPSCMMTRKVESDFKNAMKKGLKYGKLSLPTYRDTNPLLIHIDYVRLRSTNPHLDNGLYHNYKNHTEFLEHLYDENLELFIKFANKITFKIILGNPHKSSELRSVFKNIFEDCYHIQGSSIEIEKNKIILNMSMSIPVKKIELDENIVVGVDLGMAIPAVCALNTNEYIHKSLGNYNDFIRERTKIQAQKKRMQKSLTYTNGGHGRKKKLKPLNRFKERERNWVKTYNHKISKQIIDFAIKNKAKYINLEDLSGIAKEDKDKFVLRNWSYFELQQFITYKAEKYGIIVRKIKPEYTSQKCSCCGHLEENQRINQSEFICKNPNCKNFGKIVNADYNGARNIAMSTNFVEEKETKSKPKKVA

SEQ ID NO: 290 - protein, 433 aa, synthetic construct
  REGION 1..433: note = TnpB homolog
MIQNRRQNRLILTRKIQIIPLGEKEEIDRVYKYLRDGIFYQNKAMNQYMSALYIAAIKDISKEDRKELNRLYSRVSNSKKGSAYDKSIEFAKNMNLGYVVKQVKQDFANSCKNGLLCGKVSLPTYRKNNPLLVHVNFVRLRSTNYHQDNGMYHNYESHTDFLDHLYSKDLEVFIKFANNITFKMIFGNPHKSAYLRSEIQQIFEENYKVCGSSIQIDGKKIILNLSMDIPKQELELDENIVVGVDLGLAIPAMCGLNTNDYIRQSIGSKDDFLRIRTQLQSQRRRLQKSLASTSGGHGRQKKLKPLEKLKDRERNFVKTYNHYVSKNVVDFAVKNKAKYINVEDLSGFDSNQFILRNWSFYELQQFITYKAAKYGIEVRKINPYHTSQICSCCGHWEEGQRIDQAHFKCKSCGAELNADFNASRNIAMSTDFV

SEQ ID NO: 291 - protein, 453 aa, synthetic construct
  REGION 1..453: note = TnpB homolog
MTYLSLAVKVMKYQIVCPVNVEWKVFETYLRTLSYQSRTIGNRTIQKIWEFDNLSLKHFKETGEYPSAQQLYGCTQKTISGYIYDQLKEEYKDINKANMSTTIQKTLKNWNSRKKEIWRGEMSIPSFRSDLPIDIHGNSIQLIKEKGGDYIASVSLFSSKFIKENDLPNGKILMKLSTRKQNSMKVILDRLINSTYSKGACMLHKHKKKWYLSITYKSNIKEELKFDEDLIMGIDMGKINVLYFAFNKSLVRGAISGEEIEAFRKKIEHRRISLLRQGKYCSGNRIGKGREKRIKPIDVLNDKVAKFRNATNHKYANYIVQQCLKYNCGTIQLEDLKGISKEQTFLKNWTYFDLQEKIKNQANQYGVKVVKIDPSYTSQRCSECGYIHKDNRQDQSTFECLQCSFKAHADYNAAKNISVYTIEKVIQKQLELQEKLNLTKYKEQYIEQIKNIN

SEQ ID NO: 292 - protein, 450 aa, synthetic construct
  REGION 1..450: note = TnpB homolog
MSLAVKVMKYQIVCPVNVEWKVFETYLRTLSYQSRTIGNRTIQKIWEFDNLSLKHFKETGEYPSAQQLYGCTQKTISGYIYDQLKEEYKDINKANMSTTIQKTLKNWNSRKKEIWRGEMSIPSFRSDLPIDIHGNSIQLIKEKGGDYIASVSLFSSKFIKENDLPNGKILMKLSTRKQNSMKVILDRLINSTYSKGACMLHKHKKKWYLSITYKSNIKEELKFDEDLIMGIDMGKINVLYFAFNKSLVRGAISGEEIEAFRKKIEHRRISLLRQGKYCSGNRIGKGREKRIKPIDVLNDKVAKFRNATNHKYANYIVQQCLKYNCGTIQLEDLKGISKEQTFLKNWTYFDLQEKIKNQANQYGVKVVKIDPSYTSQRCSECGYIHKDNRQDQSTFECLQCSFKAHADYNAAKNISVYTIEKVIQKQLELQEKLNLTKYKEQYIEQIKNIN

SEQ ID NO: 293 - protein, 399 aa, synthetic construct
  REGION 1..399: note = TnpB homolog
MGLNHAITEWHLYERERARHYRETKENLPAEERKKTWNRIYSEVRGLMKTASSGMASMVTRTAITRYQNSLKDIRSLKQSVPSYRLGHPILLREGGGETKLWRDNGNYMFRATLRNRSNEPTRLTFLLDTFKLEKSKKAVLDRVISGEYKLGACQVAQDRRKRWFTRIAYSFPRPELKKDTSICVGVDLGLACPFYCAVNNGHDRLSCNEALIVERFRWQIRRRRRAFQNSLKFSNRGGHGRNKALAPLEKLAEKEINFRDTKYHQYTSRIIEFALKQNAGVIQIEGLEGFRASQQGILRDWAIADFHSKLKYKAEHAGIEVREIDARYTSQRCSECGNINEANRQSQSDFLCTVCGYKTHADYNAARNISIVGIEKIIAEEIARKGLAEQEAQDVPQG

SEQ ID NO: 294 - protein, 249 aa, synthetic construct
  source 1..249: note = N-term 249aa extension
MVSKGEELFTGVVPILVELDGDVNGHKFSVSGEGEGDATYGKLTLKFICTTGKLPVPWPTLVTTLTYGVQCFSRYPDHMKQHDFFKSAMPEGYVQERTIFFKDDGNYKTRAEVKFEGDTLVNRIELKGIDFKEDGNILGHKLEYNYNSHNVYIMADKQKNGIKVNFKIRHNIEDGSVQLADHYQQNTPIGDGPVLLPDNHYLSTQSALSKDPNEKRDHMVLLEFVTAAGITLGMDELYKSGLRSRAQAL

SEQ ID NO: 295 - protein, 248 aa, synthetic construct
  source 1..248: note = C-term 248aa extension
RARDPPVATMVSKGEELFTGVVPILVELDGDVNGHKFSVSGEGEGDATYGKLTLKFICTTGKLPVPWPTLVTTLTYGVQCFSRYPDHMKQHDFFKSAMPEGYVQERTIFFKDDGNYKTRAEVKFEGDTLVNRIELKGIDFKEDGNILGHKLEYNYNSHNVYIMADKQKNGIKVNFKIRHNIEDGSVQLADHYQQNTPIGDGPVLLPDNHYLSTQSALSKDPNEKRDHMVLLEFVTAAGITLGMDELYK

SEQ ID NO: 296 - DNA, 27 bp, synthetic construct
  source 1..27: mol_type = other DNA; note = Target sequence in Fig. 2
tttagagggagacacaagttgataggg

SEQ ID NO: 297 - protein, 1367 aa, synthetic construct
  source 1..1367: note = Cas9 protein
DKKYSIGLDIGTNSVGWAVITDEYKVPSKKFKVLGNTDRHSIKKNLIGALLFDSGETAEATRLKRTARRRYTRRKNRICYLQEIFSNEMAKVDDSFFHRLEESFLVEEDKKHERHPIFGNIVDEVAYHEKYPTIYHLRKKLVDSTDKADLRLIYLALAHMIKFRGHFLIEGDLNPDNSDVDKLFIQLVQTYNQLFEENPINASGVDAKAILSARLSKSRRLENLIAQLPGEKKNGLFGNLIALSLGLTPNFKSNFDLAEDAKLQLSKDTYDDDLDNLLAQIGDQYADLFLAAKNLSDAILLSDILRVNTEITKAPLSASMIKRYDEHHQDLTLLKALVRQQLPEKYKEIFFDQSKNGYAGYIDGGASQEEFYKFIKPILEKMDGTEELLVKLNREDLLRKQRTFDNGSIPHQIHLGELHAILRRQEDFYPFLKDNREKIEKILTFRIPYYVGPLARGNSRFAWMTRKSEETITPWNFEEVVDKGASAQSFIERMTNFDKNLPNEKVLPKHSLLYEYFTVYNELTKVKYVTEGMRKPAFLSGEQKKAIVDLLFKTNRKVTVKQLKEDYFKKIECFDSVEISGVEDRFNASLGTYHDLLKIIKDKDFLDNEENEDILEDIVLTLTLFEDREMIEERLKTYAHLFDDKVMKQLKRRRYTGWGRLSRKLINGIRDKQSGKTILDFLKSDGFANRNFMQLIHDDSLTFKEDIQKAQVSGQGDSLHEHIANLAGSPAIKKGILQTVKVVDELVKVMGRHKPENIVIEMARENQTTQKGQKNSRERMKRIEEGIKELGSQILKEHPVENTQLQNEKLYLYYLQNGRDMYVDQELDINRLSDYDVDHIVPQSFLKDDSIDNKVLTRSDKNRGKSDNVPSEEVVKKMKNYWRQLLNAKLITQRKFDNLTKAERGGLSELDKAGFIKRQLVETRQITKHVAQILDSRMNTKYDENDKLIREVKVITLKSKLVSDFRKDFQFYKVREINNYHHAHDAYLNAVVGTALIKKYPKLESEFVYGDYKVYDVRKMIAKSEQEIGKATAKYFFYSNIMNFFKTEITLANGEIRKRPLIETNGETGEIVWDKGRDFATVRKVLSMPQVNIVKKTEVQTGGFSKESILPKRNSDKLIARKKDWDPKKYGGFDSPTVAYSVLVVAKVEKGKSKKLKSVKELLGITIMERSSFEKNPIDFLEAKGYKEVKKDLIIKLPKYSLFELENGRKRMLASAGELQKGNELALPSKYVNFLYLASHYEKLKGSPEDNEQKQLFVEQHKHYLDEIIEQISEFSKRVILADANLDKVLSAYNKHRDKPIREQAENIIHLFTLTNLGAPAAFKYFDTTIDRKRYTSTKEVLDATLIHQSITGLYETRIDLSQLGGD

SEQ ID NO: 298 - protein, 1306 aa, synthetic construct
  source 1..1306: note = Cas12a protein
TQFEGFTNLYQVSKTLRFELIPQGKTLKHIQEQGFIEEDKARNDHYKELKPIIDRIYKTYADQCLQLVQLDWENLSAAIDSYRKEKTEETRNALIEEQATYRNAIHDYFIGRTDNLTDAINKRHAEIYKGLFKAELFNGKVLKQLGTVTTTEHENALLRSFDKFTTYFSGFYENRKNVFSAEDISTAIPHRIVQDNFPKFKENCHIFTRLITAVPSLREHFENVKKAIGIFVSTSIEEVFSFPFYNQLLTQTQIDLYNQLLGGISREAGTEKIKGLNEVLNLAIQKNDETAHIIASLPHRFIPLFKQILSDRNTLSFILEEFKSDEEVIQSFCKYKTLLRNENVLETAEALFNELNSIDLTHIFISHKKLETISSALCDHWDTLRNALYERRISELTGKITKSAKEKVQRSLKHEDINLQEIISAAGKELSEAFKQKTSEILSHAHAALDQPLPTTLKKQEEKEILKSQLDSLLGLYHLLDWFAVDESNEVDPEFSARLTGIKLEMEPSLSFYNKARNYATKKPYSVEKFKLNFQMPTLASGWDVNKEKNNGAILFVKNGLYYLGIMPKQKGRYKALSFEPTEKTSEGFDKMYYDYFPDAAKMIPKCSTQLKAVTAHFQTHTTPILLSNNFIEPLEITKEIYDLNNPEKEPKKFQTAYAKKTGDQKGYREALCKWIDFTRDFLSKYTKTTSIDLSSLRPSSQYKDLGEYYAELNPLLYHISFQRIAEKEIMDAVETGKLYLFQIYNKDFAKGHHGKPNLHTLYWTGLFSPENLAKTSIKLNGQAELFYRPKSRMKRMAHRLGEKMLNKKLKDQKTPIPDTLYQELYDYVNHRLSHDLSDEARALLPNVITKEVSHEIIKDRRFTSDKFFFHVPITLNYQAANSPSKFNQRVNAYLKEHPETPIIGIDRGERNLIYITVIDSTGKILEQRSLNTIQQFDYQKKLDNREKERVAARQAWSVVGTIKDLKQGYLSQVIHEIVDLMIHYQAVVVLENLNFGFKSKRTGIAEKAVYQQFEKMLIDKLNCLVLKDYPAEKVGGVLNPYQLTDQFTSFAKMGTQSGFLFYVPAPYTSKIDPLTGFVDPFVWKTIKNHESRKHFLEGFDFLHYDVKTGDFILHFKMNRNLSFQRGLPGFMPAWDIVFEKNETQFDAKGTPFIAGKRIVPVIENHRFTGRYRDLYPANELIALLEEKGIVFRDGSNILPKLLENDDSHAIDTMVALIRSVLQMRNSNAATGEDYINSPVRDLNGVCFDSRFQNPEWPMDADANGAYHIALKGQLLLNHLKESKDLKLQNGISNQDWLAYIQELRN

SEQ ID NO: 299 - RNA, 102 nt, synthetic construct
  source 1..102: mol_type = other RNA; note = Cas9 gRNA
gagggagacacaagttgatagttttagagctagaaatagcaagttaaaataaggctagtccgttatcaacttgaaaaagtggcaccgagtcggtgctttttt

SEQ ID NO: 300 - RNA, 76 nt, synthetic construct
  source 1..76: mol_type = other RNA; note = Cas9 gRNA scaffold
gttttagagctagaaatagcaagttaaaataaggctagtccgttatcaacttgaaaaagtggcaccgagtcggtgc

SEQ ID NO: 301 - RNA, 40 nt, synthetic construct
  source 1..40: mol_type = other RNA; note = Cas12a gRNA
taatttctactcttgtagatgagggagacacaagttgata

SEQ ID NO: 302 - RNA, 20 nt, synthetic construct
  source 1..20: mol_type = other RNA; note = Cas12a crRNA
taatttctactcttgtagat